European Patent Specification EP 2 866 826 B1, published August 6, 2025. Title: Combination for treating an inflammatory disorder. Applicant: Arthrogen B.V. The sequence listing filed with the application follows.

SEQUENCE LISTING (57 sequences)

SEQ ID NO: 1 - protein, 510 aa, Artificial
  CD39 derived from homo sapiens
MEDTKESNVKTFCSKNILAILGFSSIIAVIALLAVGLTQNKALPENVKYGIVLDAGSSHTSLYIYKWPAEKENDTGVVHQVEECRVKGPGISKFVQKVNEIGIYLTDCMERAREVIPRSQHQETPVYLGATAGMRLLRMESEELADRVLDVVERSLSNYPFDFQGARIITGQEEGAYGWITINYLLGKFSQKTRWFSIVPYETNNQETFGALDLGGASTQVTFVPQNQTIESPDNALQFRLYGKDYNVYTHSFLCYGKDQALWQKLAKDIQVASNEILRDPCFHPGYKKVVNVSDLYKTPCTKRFEMTLPFQQFEIQGIGNYQQCHQSILELFNTSYCPYSQCAFNGIFLPPLQGDFGAFSAFYFVMKFLNLTSEKVSQEKVTEMMKKFCAQPWEEIKTSYAGVKEKYLSEYCFSGTYILSLLLQGYHFTADSWEHIHFIGKIQGSDAGWTLGYMLNLTNMIPAEQPLSTPLSHSTYVFLMVLFSLVLFTVAIIGLLIFHKPSYFWKDMV

SEQ ID NO: 2 - DNA, 1533 bp, Artificial
  CD39 derived from homo sapiens
atggaggacaccaaggagagcaacgtgaagaccttctgcagcaagaacatcctggccatcctgggcttcagcagcatcatcgccgtgatcgccctgctggccgtgggcctgacccagaacaaggccctgcccgagaacgtgaagtacggcatcgtgctggacgccggcagcagccacaccagcctgtacatctacaagtggcccgccgagaaggagaacgacaccggcgtggtgcaccaggtggaggagtgcagagtgaagggccccggcatcagcaagttcgtgcagaaggtgaacgagatcggcatctacctgaccgactgcatggagagagccagagaggtgatccccagaagccagcaccaggagacccccgtgtacctgggcgccaccgccggcatgagactgctgagaatggagagcgaggagctggccgacagagtgctggacgtggtggagagaagcctgagcaactaccccttcgacttccagggcgccagaatcatcaccggccaggaggagggcgcctacggctggatcaccatcaactacctgctgggcaagttcagccagaagaccagatggttcagcatcgtgccctacgagaccaacaaccaggagaccttcggcgccctggacctgggcggcgccagcacccaggtgaccttcgtgccccagaaccagaccatcgagagccccgacaacgccctgcagttcagactgtacggcaaggactacaacgtgtacacccacagcttcctgtgctacggcaaggaccaggccctgtggcagaagctggccaaggacatccaggtggccagcaacgagatcctgagagacccctgcttccaccccggctacaagaaggtggtgaacgtgagcgacctgtacaagaccccctgcaccaagagattcgagatgaccctgcccttccagcagttcgagatccagggcatcggcaactaccagcagtgccaccagagcatcctggagctgttcaacaccagctactgcccctacagccagtgcgccttcaacggcatcttcctgccccccctgcagggcgacttcggcgccttcagcgccttctacttcgtgatgaagttcctgaacctgaccagcgagaaggtgagccaggagaaggtgaccgagatgatgaagaagttctgcgcccagccctgggaggagatcaagaccagctacgccggcgtgaaggagaagtacctgagcgagtactgcttcagcggcacctacatcctgagcctgctgctgcagggctaccacttcaccgccgacagctgggagcacatccacttcatcggcaagatccagggcagcgacgccggctggaccctgggctacatgctgaacctgaccaacatgatccccgccgagcagcccctgagcacccccctgagccacagcacctacgtgttcctgatggtgctgttcagcctggtgctgttcaccgtggccatcatcggcctgctgatcttccacaagcccagctacttctggaaggacatggtgtga

SEQ ID NO: 3 - protein, 574 aa, Artificial [sequence omitted]

SEQ ID NO: 4 - DNA, 1725 bp, Artificial
  CD73 derived from homo sapiens
atgtgccccagagccgccagagcccccgccaccctgctgctggccctgggcgccgtgctgtggcccgccgccggcgcctgggagctgaccatcctgcacaccaacgacgtgcacagcagactggagcagaccagcgaggacagcagcaagtgcgtgaacgccagcagatgcatgggcggcgtggccagactgttcaccaaggtgcagcagatcagaagagccgagcccaacgtgctgctgctggacgccggcgaccagtaccagggcaccatctggttcaccgtgtacaagggcgccgaggtggcccacttcatgaacgccctgagatacgacgccatggccctgggcaaccacgagttcgacaacggcgtggagggcctgatcgagcccctgctgaaggaggccaagttccccatcctgagcgccaacatcaaggccaagggccccctggccagccagatcagcggcctgtacctgccctacaaggtgctgcccgtgggcgacgaggtggtgggcatcgtgggctacaccagcaaggagacccccttcctgagcaaccccggcaccaacctggtgttcgaggacgagatcaccgccctgcagcccgaggtggacaagctgaagaccctgaacgtgaacaagatcatcgccctgggccacagcggcttcgagatggacaagctgatcgcccagaaggtgagaggcgtggacgtggtggtgggcggccacagcaacaccttcctgtacaccggcaacccccccagcaaggaggtgcccgccggcaagtaccccttcatcgtgaccagcgacgacggcagaaaggtgcccgtggtgcaggcctacgccttcggcaagtacctgggctacctgaagatcgagttcgacgagagaggcaacgtgatcagcagccacggcaaccccatcctgctgaacagcagcatccccgaggaccccagcatcaaggccgacatcaacaagtggagaatcaagctggacaactacagcacccaggagctgggcaagaccatcgtgtacctggacggcagcagccagagctgcagattcagagagtgcaacatgggcaacctgatctgcgacgccatgatcaacaacaacctgagacacgccgacgagaccttctggaaccacgtgagcatgtgcatcctgaacggcggcggcatcagaagccccatcgacgagagaaacaacggcaccatcacctgggagaacctggccgccgtgctgcccttcggcggcaccttcgacctggtgcagctgaagggcagcaccctgaagaaggccttcgagcacagcgtgcacagatacggccagagcaccggcgagttcctgcaggtgggcggcatccacgtggtgtacgacctgagcagaaagcccggcgacagagtggtgaagctggacgtgctgtgcaccaagtgcagagtgcccagctacgaccccctgaagatggacgaggtgtacaaggtgatcctgcccaacttcctggccaacggcggcgacggcttccagatgatcaaggacgagctgctgagacacgacagcggcgaccaggacatcaacgtggtgagcacctacatcagcaagatgaaggtgatctaccccgccgtggagggcagaatcaagttcagcaccggcagccactgccacggcagcttcagcctgatcttcctgagcctgtgggccgtgatcttcgtgctgtaccagtga

SEQ ID NO: 5 - protein, 513 aa, Artificial
  CD39 derived from mus musculus
MSRMEDIKDSKVKRFCSKNILIILGFTSILAVIALIAVGLTQNKPLPENVKYGIVLDAGSSHTNLYIYKWPAEKENDTGVVQQLEECQVKGPGISKYAQKTDEIGAYLAECMELSTELIPTSKHHQTPVYLGATAGMRLLRMESEQSADEVLAAVSTSLKSYPFDFQGAKIITGQEEGAYGWITINYLLGRFTQEQSWLSLISDSQKQETFGALDLGGASTQITFVPQNSTIESPENSLQFRLYGEDYTVYTHSFLCYGKDQALWQKLAKDIQVSSGGVLKDPCFNPGYEKVVNVSELYGTPCTKRFEKKLPFDQFRIQGTGDYEQCHQSILELFNNSHCPYSQCAFNGVFLPPLHGSFGAFSAFYFVMDFFKKVAKNSVISQEKMTEITKNFCSKSWEETKTSYPSVKEKYLSEYCFSGAYILSLLQGYNFTDSSWEQIHFMGKIKDSNAGWTLGYMLNLTNMIPAEQPLSPPLPHSTYIGLMVLFSLLLVAVAITGLFIYSKPSYFWKEAV

SEQ ID NO: 6 - DNA, 1542 bp, Artificial
  CD39 derived from mus musculus, codon optimized
atgagccgcatggaggacatcaaagactcaaaagtgaaaagattctgctcaaaaaacattctcatcattctggggtttacatcaattctcgctgtgatcgcactgattgccgtcggcctcactcagaacaagcccctgcctgagaacgtgaagtacggaatcgtcctggacgctgggagctcccacaccaatctgtacatctacaagtggccagcagagaaagaaaacgatacaggcgtggtccagcagctggaggaatgccaggtgaagggtcccggcatctccaagtacgcccagaaaacagacgagattggagcttatctggcagagtgtatggaactgagcacagaactcatccccacttccaagcaccatcagacacccgtgtacctgggtgcaactgcaggaatgcgactgctccgcatggagtcagaacagagcgccgacgaggtgctggcagctgtcagtacttcactcaaatcttatccattcgattttcagggtgccaagatcattaccggccaggaggaaggagcttacgggtggatcactattaactatctgctcgggcggttcacccaggagcagtcctggctgtctctcatcagcgactcccagaagcaggaaaccttcggcgctctggatctcggcggagcaagcacccagatcacatttgtgccacagaatagcacaattgagtcccccgaaaactctctgcagttccgcctctacggggaggactacaccgtgtacacccactcctttctgtgctatggcaaggaccaggccctgtggcagaagctcgctaaagatatccaggtgtctagtgggggtgtcctgaaagatccctgcttcaatcctggttacgagaaggtggtcaacgtgtctgaactgtatggaacaccatgtactaagaggttcgagaagaaactgcccttcgaccagtttcgaatccagggaaccggggattacgagcagtgtcaccagagcattctggaactcttcaacaatagccattgcccatattcccagtgtgccttcaacggagtgtttctgccccctctccacggttctttcggcgcctttagtgctttctactttgtgatggacttctttaagaaagtggctaagaatagtgtcatctcacaggagaagatgaccgaaatcacaaagaacttctgctctaagagttgggaggaaaccaagacaagctacccctccgtgaaggagaaatacctgtcagaatattgttttagcggtgcctacatcctgtccctgctccagggctataatttcaccgactcaagctgggagcagatccactttatgggcaagatcaaggattctaacgccggatggaccctggggtacatgctgaatctcacaaacatgatcccagctgagcagccactgtccccaccactccctcattctacctatattggcctgatggtgctcttctccctgctcctggtggctgtcgcaatcacaggactgttcatctactctaagccaagttatttttggaaagaggcagtgtga

SEQ ID NO: 7 - protein, 574 aa, Artificial
  CD73 derived from mus  musculus
MRPAAAKVPKWLLLALSALLPQWPAASAWELTILHTNDVHSRLEQTSDDSTKCLNASLCVGGVARLFTKVQQIRKEEPNVLFLDAGDQYQGTIWFTVYKGLEVAHFMNILGYDAMALGNHEFDNGVEGLIDPLLRNVKFPILSANIKARGPLAHQISGLFLPSKVLSVGGEVVGIVGYTSKETPFLSNPGTNLVFEDEISALQPEVDKLKTLNVNKIIALGHSGFEMDKLIAQKVRGVDIVVGGHSNTFLYTGNPPSKEVPAGKYPFIVTADDGRQVPVVQAYAFGKYLGYLKVEFDDKGNVITSYGNPILLNSSIPEDATIKADINQWRIKLDNYSTQELGRTIVYLDGSTQTCRFRECNMGNLICDAMINNNLRHPDEMFWNHVSMCIVNGGGIRSPIDEKNNGTITWENLAAVLPFGGTFDLVQLKGSTLKKAFEHSVHRYGQSTGEFLQVGGIHVVYDINRKPWNRVVQLEVLCTKCRVPIYEPLEMDKVYKVTLPSYLANGGDGFQMIKDELLKHDSGDQDISVVSEYISKMKVVYPAVEGRIKFSAASHYQGSFPLVILSFWAMILIL

SEQ ID NO: 8 - DNA, 1725 bp, Artificial
  CD73 derived from mus musculus, codon optimized
atgaggcctgcagccgctaaggtgccaaaatggctcctgctcgcactgtccgccctgctccctcagtggccagcagcctctgcttgggagctgactatcctccacaccaatgatgtgcatagtagactggaacagacctcagacgatagcacaaagtgcctgaacgccagcctgtgcgtgggaggagtcgcaagactgttcaccaaggtgcagcagatccggaaagaggaacctaatgtcctgtttctcgacgcaggcgaccagtaccagggcacaatctggttcaccgtgtacaagggactggaggtcgctcactttatgaacattctgggttacgacgccatggctctcggcaatcatgagttcgacaacggagtggaagggctgatcgatcctctgctccggaatgtgaaatttccaatcctgtcagctaacattaaggcacgaggtcctctggcacaccagatcagcggactgttcctcccaagtaaagtgctgtcagtcgggggcgaggtggtcggtattgtgggctacacctctaaggaaacacccttcctgagtaatcctggcacaaacctcgtgtttgaggacgaaatctctgccctgcagcctgaggtggataagctgaaaactctcaatgtcaacaagatcattgcactgggacacagcgggttcgaaatggacaagctgatcgcccagaaagtgagaggggtcgatattgtggtcggcggacatagtaatactttcctgtacaccggaaaccctccatcaaaggaggtgccagctgggaaatatccctttatcgtgaccgcagacgatggccggcaggtcccagtggtccaggcatacgccttcggcaagtacctgggctatctcaaagtggagtttgacgataagggaaacgtcatcacaagctatgggaatcccatcctgctcaactcctctattcctgaagacgccactatcaaagctgatattaatcagtggaggatcaagctggacaactactccactcaggagctgggaagaaccatcgtgtacctggatgggtctactcagacctgcaggttcagagaatgtaatatgggcaacctgatctgcgacgccatgattaacaataacctgcgacaccccgatgagatgttttggaatcatgtgagcatgtgcatcgtcaacgggggtggcatcaggtcccccattgacgagaagaataacggaacaattacttgggaaaacctggctgcagtgctccctttcggagggacatttgatctggtccagctcaaggggtccactctgaagaaagccttcgagcactcagtgcatcgctacggacagagcaccggggaatttctgcaagtgggtggcatccacgtggtctatgacattaatcgaaaaccctggaacagggtggtccagctggaggtgctctgcactaagtgtcgagtccctatctacgagccactggaaatggacaaggtgtacaaagtcaccctgcctagctatctcgccaacggaggggatggattccagatgattaaggacgagctgctcaaacatgattctggggaccaggatatctccgtggtctctgagtacattagtaagatgaaagtggtctatcctgctgtggaaggcaggatcaagttcagtgccgcttcacattaccagggttcttttccactcgtgattctctctttttgggctatgattctgattctctga

SEQ ID NO: 9 - protein, 464 aa, Artificial
  soluble CD39 derived from mus musculus
MPSSVSWGILLLAGLCCLVPVSLAETQNKPLPENVKYGIVLDAGSSHTNLYIYKWPAEKENDTGVVQQLEECQVKGPGISKYAQKTDEIGAYLAECMELSTELIPTSKHHQTPVYLGATAGMRLLRMESEQSADEVLAAVSTSLKSYPFDFQGAKIITGQEEGAYGWITINYLLGRFTQEQSWLSLISDSQKQETFGALDLGGASTQITFVPQNSTIESPENSLQFRLYGEDYTVYTHSFLCYGKDQALWQKLAKDIQVSSGGVLKDPCFNPGYEKVVNVSELYGTPCTKRFEKKLPFDQFRIQGTGDYEQCHQSILELFNNSHCPYSQCAFNGVFLPPLHGSFGAFSAFYFVMDFFKKVAKNSVISQEKMTEITKNFCSKSWEETKTSYPSVKEKYLSEYCFSGAYILSLLQGYNFTDSSWEQIHFMGKIKDSNAGWTLGYMLNLTNMIPAEQPLSPPLPHST

SEQ ID NO: 10 - DNA, 1395 bp, Artificial
  soluble CD39 derived from mus musculus, codon optimized
atgccttcctccgtctcatggggtatcctcctgctcgctgggctgtgctgcctggtgcctgtctcactcgccgaaactcagaacaagccactgcccgagaacgtgaagtacggcatcgtcctggacgcaggaagctcccacacaaacctctacatctacaagtggcccgccgagaaagaaaatgatactggagtggtccagcagctggaggaatgccaggtgaagggccctggaatctccaagtacgcccagaaaaccgacgagattggggcttatctggcagagtgtatggaactgtcaacagaactcatccccacttctaaacaccatcagacccccgtgtacctgggagcaacagcaggaatgaggctgctcagaatggagtctgaacagagtgctgacgaggtgctggccgctgtctccacctctctcaagagctatcccttcgattttcagggggccaaaatcattaccggtcaggaggaaggcgcttacggatggatcactattaactatctgctcgggcgattcacccaggagcagtcatggctgagcctcatcagtgactcacagaagcaggaaactttcggcgcactggatctcggaggagcaagcactcagatcacctttgtgccacagaacagcaccattgagtcccccgaaaattctctgcagttcagactctacggcgaggactacacagtctatactcattcctttctgtgctatggaaaggaccaggctctgtggcagaagctcgcaaaagatattcaggtgtctagtgggggtgtcctgaaggatccttgcttcaacccagggtacgagaaagtggtcaacgtgagcgaactgtatggtaccccttgtacaaagcggtttgagaagaaactgccattcgaccagtttcgcatccaggggacaggcgactacgagcagtgtcaccagagcattctggaactcttcaacaatagtcattgcccatattcacagtgtgctttcaacggcgtgtttctgccacctctccacgggagcttcggtgccttttccgctttctacttcgtcatggatttctttaagaaagtggcaaagaactccgtcatctctcaggagaagatgactgaaatcaccaagaacttctgcagcaaatcctgggaggaaaccaagacaagttatccctcagtgaaggagaaatacctgtctgaatattgttttagtggcgcctacatcctgagtctgctccagggatataatttcacagactcaagctgggagcagatccacttcatgggcaagatcaaggattctaacgctgggtggactctgggttacatgctcaatctcaccaatatgattccagccgaacagccactcagccccccactcccacactcaacctga

SEQ ID NO: 11 - protein, 464 aa, Artificial
  soluble CD39 derived from homo sapiens
MPSSVSWGILLLAGLCCLVPVSLAETQNKALPENVKYGIVLDAGSSHTSLYIYKWPAEKENDTGVVHQVEECRVKGPGISKFVQKVNEIGIYLTDCMERAREVIPRSQHQETPVYLGATAGMRLLRMESEELADRVLDVVERSLSNYPFDFQGARIITGQEEGAYGWITINYLLGKFSQKTRWFSIVPYETNNQETFGALDLGGASTQVTFVPQNQTIESPDNALQFRLYGKDYNVYTHSFLCYGKDQALWQKLAKDIQVASNEILRDPCFHPGYKKVVNVSDLYKTPCTKRFEMTLPFQQFEIQGIGNYQQCHQSILELFNTSYCPYSQCAFNGIFLPPLQGDFGAFSAFYFVMKFLNLTSEKVSQEKVTEMMKKFCAQPWEEIKTSYAGVKEKYLSEYCFSGTYILSLLLQGYHFTADSWEHIHFIGKIQGSDAGWTLGYMLNLTNMIPAEQPLSTPLSHST

SEQ ID NO: 12 - DNA, 1395 bp, Artificial
  soluble CD39 derived from homo sapiens, codon optimized
atgcccagcagcgtgagctggggcatcctgctgctggccggcctgtgctgcctggtgcccgtgagcctggccgagacccagaacaaggccctgcccgagaacgtgaagtacggcatcgtgctggacgccggcagcagccacaccagcctgtacatctacaagtggcccgccgagaaggagaacgacaccggcgtggtgcaccaggtggaggagtgcagagtgaagggccccggcatcagcaagttcgtgcagaaggtgaacgagatcggcatctacctgaccgactgcatggagagagccagagaggtgatccccagaagccagcaccaggagacccccgtgtacctgggcgccaccgccggcatgagactgctgagaatggagagcgaggagctggccgacagagtgctggacgtggtggagagaagcctgagcaactaccccttcgacttccagggcgccagaatcatcaccggccaggaggagggcgcctacggctggatcaccatcaactacctgctgggcaagttcagccagaagaccagatggttcagcatcgtgccctacgagaccaacaaccaggagaccttcggcgccctggacctgggcggcgccagcacccaggtgaccttcgtgccccagaaccagaccatcgagagccccgacaacgccctgcagttcagactgtacggcaaggactacaacgtgtacacccacagcttcctgtgctacggcaaggaccaggccctgtggcagaagctggccaaggacatccaggtggccagcaacgagatcctgagagacccctgcttccaccccggctacaagaaggtggtgaacgtgagcgacctgtacaagaccccctgcaccaagagattcgagatgaccctgcccttccagcagttcgagatccagggcatcggcaactaccagcagtgccaccagagcatcctggagctgttcaacaccagctactgcccctacagccagtgcgccttcaacggcatcttcctgccccccctgcagggcgacttcggcgccttcagcgccttctacttcgtgatgaagttcctgaacctgaccagcgagaaggtgagccaggagaaggtgaccgagatgatgaagaagttctgcgcccagccctgggaggagatcaagaccagctacgccggcgtgaaggagaagtacctgagcgagtactgcttcagcggcacctacatcctgagcctgctgctgcagggctaccacttcaccgccgacagctgggagcacatccacttcatcggcaagatccagggcagcgacgccggctggaccctgggctacatgctgaacctgaccaacatgatccccgccgagcagcccctgagcacccccctgagccacagcacctga

SEQ ID NO: 13 - protein, 550 aa, Artificial
  soluble CD73 derived from mus musculus
MRPAAAKVPKWLLLALSALLPQWPAASAWELTILHTNDVHSRLEQTSDDSTKCLNASLCVGGVARLFTKVQQIRKEEPNVLFLDAGDQYQGTIWFTVYKGLEVAHFMNILGYDAMALGNHEFDNGVEGLIDPLLRNVKFPILSANIKARGPLAHQISGLFLPSKVLSVGGEVVGIVGYTSKETPFLSNPGTNLVFEDEISALQPEVDKLKTLNVNKIIALGHSGFEMDKLIAQKVRGVDIVVGGHSNTFLYTGNPPSKEVPAGKYPFIVTADDGRQVPVVQAYAFGKYLGYLKVEFDDKGNVITSYGNPILLNSSIPEDATIKADINQWRIKLDNYSTQELGRTIVYLDGSTQTCRFRECNMGNLICDAMINNNLRHPDEMFWNHVSMCIVNGGGIRSPIDEKNNGTITWENLAAVLPFGGTFDLVQLKGSTLKKAFEHSVHRYGQSTGEFLQVGGIHVVYDINRKPWNRVVQLEVLCTKCRVPIYEPLEMDKVYKVTLPSYLANGGDGFQMIKDELLKHDSGDQDISVVSEYISKMKVVYPAVEGRIKF

SEQ ID NO: 14 - DNA, 1653 bp, Artificial
  soluble CD73 derived from mus musculus, codon optimized
atgaggcctgcagccgctaaggtgccaaaatggctcctgctcgcactgtccgccctgctccctcagtggccagcagcctctgcttgggagctgactatcctccacaccaatgatgtgcatagtagactggaacagacctcagacgatagcacaaagtgcctgaacgccagcctgtgcgtgggaggagtcgcaagactgttcaccaaggtgcagcagatccggaaagaggaacctaatgtcctgtttctcgacgcaggcgaccagtaccagggcacaatctggttcaccgtgtacaagggactggaggtcgctcactttatgaacattctgggttacgacgccatggctctcggcaatcatgagttcgacaacggagtggaagggctgatcgatcctctgctccggaatgtgaaatttccaatcctgtcagctaacattaaggcacgaggtcctctggcacaccagatcagcggactgttcctcccaagtaaagtgctgtcagtcgggggcgaggtggtcggtattgtgggctacacctctaaggaaacacccttcctgagtaatcctggcacaaacctcgtgtttgaggacgaaatctctgccctgcagcctgaggtggataagctgaaaactctcaatgtcaacaagatcattgcactgggacacagcgggttcgaaatggacaagctgatcgcccagaaagtgagaggggtcgatattgtggtcggcggacatagtaatactttcctgtacaccggaaaccctccatcaaaggaggtgccagctgggaaatatccctttatcgtgaccgcagacgatggccggcaggtcccagtggtccaggcatacgccttcggcaagtacctgggctatctcaaagtggagtttgacgataagggaaacgtcatcacaagctatgggaatcccatcctgctcaactcctctattcctgaagacgccactatcaaagctgatattaatcagtggaggatcaagctggacaactactccactcaggagctgggaagaaccatcgtgtacctggatgggtctactcagacctgcaggttcagagaatgtaatatgggcaacctgatctgcgacgccatgattaacaataacctgcgacaccccgatgagatgttttggaatcatgtgagcatgtgcatcgtcaacgggggtggcatcaggtcccccattgacgagaagaataacggaacaattacttgggaaaacctggctgcagtgctccctttcggagggacatttgatctggtccagctcaaggggtccactctgaagaaagccttcgagcactcagtgcatcgctacggacagagcaccggggaatttctgcaagtgggtggcatccacgtggtctatgacattaatcgaaaaccctggaacagggtggtccagctggaggtgctctgcactaagtgtcgagtccctatctacgagccactggaaatggacaaggtgtacaaagtcaccctgcctagctatctcgccaacggaggggatggattccagatgattaaggacgagctgctcaaacatgattctggggaccaggatatctccgtggtctctgagtacattagtaagatgaaagtggtctatcctgctgtggaaggcaggatcaagttctga

SEQ ID NO: 15 - protein, 548 aa, Artificial
  soluble CD73 derived from homo sapiens
MCPRAARAPATLLLALGAVLWPAAGAWELTILHTNDVHSRLEQTSEDSSKCVNASRCMGGVARLFTKVQQIRRAEPNVLLLDAGDQYQGTIWFTVYKGAEVAHFMNALRYDAMALGNHEFDNGVEGLIEPLLKEAKFPILSANIKAKGPLASQISGLYLPYKVLPVGDEVVGIVGYTSKETPFLSNPGTNLVFEDEITALQPEVDKLKTLNVNKIIALGHSGFEMDKLIAQKVRGVDVVVGGHSNTFLYTGNPPSKEVPAGKYPFIVTSDDGRKVPVVQAYAFGKYLGYLKIEFDERGNVISSHGNPILLNSSIPEDPSIKADINKWRIKLDNYSTQELGKTIVYLDGSSQSCRFRECNMGNLICDAMINNNLRHADETFWNHVSMCILNGGGIRSPIDERNNGTITWENLAAVLPFGGTFDLVQLKGSTLKKAFEHSVHRYGQSTGEFLQVGGIHVVYDLSRKPGDRVVKLDVLCTKCRVPSYDPLKMDEVYKVILPNFLANGGDGFQMIKDELLRHDSGDQDINVVSTYISKMKVIYPAVEGRIKF

SEQ ID NO: 16 - DNA, 1647 bp, Artificial
  soluble CD73 derived from homo sapiens, codon optimized
atgtgccccagagccgccagagcccccgccaccctgctgctggccctgggcgccgtgctgtggcccgccgccggcgcctgggagctgaccatcctgcacaccaacgacgtgcacagcagactggagcagaccagcgaggacagcagcaagtgcgtgaacgccagcagatgcatgggcggcgtggccagactgttcaccaaggtgcagcagatcagaagagccgagcccaacgtgctgctgctggacgccggcgaccagtaccagggcaccatctggttcaccgtgtacaagggcgccgaggtggcccacttcatgaacgccctgagatacgacgccatggccctgggcaaccacgagttcgacaacggcgtggagggcctgatcgagcccctgctgaaggaggccaagttccccatcctgagcgccaacatcaaggccaagggccccctggccagccagatcagcggcctgtacctgccctacaaggtgctgcccgtgggcgacgaggtggtgggcatcgtgggctacaccagcaaggagacccccttcctgagcaaccccggcaccaacctggtgttcgaggacgagatcaccgccctgcagcccgaggtggacaagctgaagaccctgaacgtgaacaagatcatcgccctgggccacagcggcttcgagatggacaagctgatcgcccagaaggtgagaggcgtggacgtggtggtgggcggccacagcaacaccttcctgtacaccggcaacccccccagcaaggaggtgcccgccggcaagtaccccttcatcgtgaccagcgacgacggcagaaaggtgcccgtggtgcaggcctacgccttcggcaagtacctgggctacctgaagatcgagttcgacgagagaggcaacgtgatcagcagccacggcaaccccatcctgctgaacagcagcatccccgaggaccccagcatcaaggccgacatcaacaagtggagaatcaagctggacaactacagcacccaggagctgggcaagaccatcgtgtacctggacggcagcagccagagctgcagattcagagagtgcaacatgggcaacctgatctgcgacgccatgatcaacaacaacctgagacacgccgacgagaccttctggaaccacgtgagcatgtgcatcctgaacggcggcggcatcagaagccccatcgacgagagaaacaacggcaccatcacctgggagaacctggccgccgtgctgcccttcggcggcaccttcgacctggtgcagctgaagggcagcaccctgaagaaggccttcgagcacagcgtgcacagatacggccagagcaccggcgagttcctgcaggtgggcggcatccacgtggtgtacgacctgagcagaaagcccggcgacagagtggtgaagctggacgtgctgtgcaccaagtgcagagtgcccagctacgaccccctgaagatggacgaggtgtacaaggtgatcctgcccaacttcctggccaacggcggcgacggcttccagatgatcaaggacgagctgctgagacacgacagcggcgaccaggacatcaacgtggtgagcacctacatcagcaagatgaaggtgatctaccccgccgtggagggcagaatcaagttctga

SEQ ID NO: 17 - protein, 1009 aa, Artificial
  soluble CD73-CD39 fusion derived from mus musculus
MPSSVSWGILLLAGLCCLVPVSLAEWELTILHTNDVHSRLEQTSDDSTKCLNASLCVGGVARLFTKVQQIRKEEPNVLFLDAGDQYQGTIWFTVYKGLEVAHFMNILGYDAMALGNHEFDNGVEGLIDPLLRNVKFPILSANIKARGPLAHQISGLFLPSKVLSVGGEVVGIVGYTSKETPFLSNPGTNLVFEDEISALQPEVDKLKTLNVNKIIALGHSGFEMDKLIAQKVRGVDIVVGGHSNTFLYTGNPPSKEVPAGKYPFIVTADDGRQVPVVQAYAFGKYLGYLKVEFDDKGNVITSYGNPILLNSSIPEDATIKADINQWRIKLDNYSTQELGRTIVYLDGSTQTCRFRECNMGNLICDAMINNNLRHPDEMFWNHVSMCIVNGGGIRSPIDEKNNGTITWENLAAVLPFGGTFDLVQLKGSTLKKAFEHSVHRYGQSTGEFLQVGGIHVVYDINRKPWNRVVQLEVLCTKCRVPIYEPLEMDKVYKVTLPSYLANGGDGFQMIKDELLKHDSGDQDISVVSEYISKMKVVYPAVEGRIKFASGGGAGGGAGGGAGGGAGGGTGTQNKPLPENVKYGIVLDAGSSHTNLYIYKWPAEKENDTGVVQQLEECQVKGPGISKYAQKTDEIGAYLAECMELSTELIPTSKHHQTPVYLGATAGMRLLRMESEQSADEVLAAVSTSLKSYPFDFQGAKIITGQEEGAYGWITINYLLGRFTQEQSWLSLISDSQKQETFGALDLGGASTQITFVPQNSTIESPENSLQFRLYGEDYTVYTHSFLCYGKDQALWQKLAKDIQVSSGGVLKDPCFNPGYEKVVNVSELYGTPCTKRFEKKLPFDQFRIQGTGDYEQCHQSILELFNNSHCPYSQCAFNGVFLPPLHGSFGAFSAFYFVMDFFKKVAKNSVISQEKMTEITKNFCSKSWEETKTSYPSVKEKYLSEYCFSGAYILSLLQGYNFTDSSWEQIHFMGKIKDSNAGWTLGYMLNLTNMIPAEQPLSPPLPHST

SEQ ID NO: 18 - DNA, 3030 bp, Artificial
  soluble CD73-CD39 fusion derived from mus musculus, codon optimized
atgcctagtagcgtgagttgggggattctgctgctggctggtctctgctgcctggtgcccgtgagtctcgccgagtgggaactgacaatcctgcacaccaatgacgtgcatagtcggctcgagcagacatcagacgatagcactaagtgcctgaacgccagcctgtgcgtgggaggagtcgcaagactgttcacaaaggtgcagcagatccggaaagaggaacctaatgtcctgtttctcgacgctggcgatcagtaccagggaacaatctggttcaccgtgtacaagggcctggaggtcgcacactttatgaacattctggggtacgacgctatggcactcggtaatcatgagttcgacaacggggtggaaggtctgatcgatcctctgctccggaatgtgaaatttccaatcctgtcagcaaacattaaggcacgaggaccactggcacaccagatcagcggtctgttcctcccctccaaagtgctgtctgtcgggggcgaggtggtcggcattgtgggatacacctctaaggaaacacccttcctgagtaatcctggcactaacctcgtgtttgaggacgaaatcagtgctctgcagcccgaggtggataagctgaaaaccctcaatgtcaacaagatcattgctctggggcactctggtttcgaaatggacaagctgatcgcacagaaagtgagaggcgtcgatattgtggtcggcggacatagtaatactttcctgtacaccggcaaccccccttcaaaggaggtgccagccggaaaatatccctttatcgtgaccgctgacgatggacggcaggtccctgtggtccaggcctacgctttcggcaagtacctgggatatctcaaagtggagtttgacgataagggcaacgtcattacatcctatggaaatcccatcctgctcaacagctccattcctgaagacgctactatcaaagcagatattaatcagtggaggatcaagctggacaactactccactcaggagctggggagaaccatcgtgtacctggatggctctacccagacatgcaggttcagagaatgtaatatgggcaacctgatctgcgacgccatgattaacaataacctgcgacacccagatgagatgttttggaatcatgtgagcatgtgcatcgtcaacgggggtggcatcaggtcccctattgacgagaagaataacggaactattacctgggaaaacctggccgctgtgctcccattcggagggacatttgatctggtgcagctcaaggggagcactctgaagaaagccttcgagcactcagtgcatcgctacgggcagagcacaggtgaatttctgcaagtgggtggcatccacgtggtctatgacattaatcgaaaaccatggaacagggtggtccagctggaggtgctctgcaccaagtgtcgagtcccaatctacgagcccctggaaatggacaaggtgtacaaagtcacactgcccagctatctcgccaacggaggggatggattccagatgattaaggacgagctgctcaaacatgattctggggaccaggatatctccgtggtctctgagtacattagtaagatgaaagtggtctatccagctgtggaaggcaggatcaagttcgctagcggtggaggagcaggaggtggagctggagggggtgcaggcggaggggccggtggcggaaccggtactcagaacaagcctctgccagagaacgtgaagtacgggatcgtcctggacgccggttctagtcacaccaatctctacatctacaagtggcccgctgagaaagaaaacgatacaggcgtggtccagcagctggaggaatgccaggtgaaggggcctggtatctctaagtacgcccagaaaaccgacgagattggagcttatctggcagagtgtatggaactgtccaccgaactcatcccaacatctaagcaccatcagacacccgtgtacctgggagcaactgcaggaatgcgactgctccgcatggagagtgaacagtcagctgacgaggtgctggcagccgtcagtacttcactcaaaagctatcccttcgattttcagggcgcaaagatcattaccggacaggaggaaggcgcctacggatggatcactattaactatctgctcgggaggttcacccaggagcagagctggctgtccctcatcagcgactcccagaagcaggaaacattcggcgctctggatctcgggggtgcatctactcagatcacctttgtgcctcagaatagtactattgagtcaccagaaaacagcctgcagttcagactctacggcgaggactacacagtgtatactcacagctttctgtgctatggaaaggaccaggccctgtggcagaagctcgctaaagatatccaggtgtcaagcggcggagtcctgaaagatccttgcttcaatccagggtacgagaaggtggtcaacgtgtccgaactgtatggcaccccctgtacaaagaggttcgagaagaaactgcctttcgaccagtttcgaatccagggcaccggagattacgagcagtgtcaccagtctattctggaactcttcaataactcccattgcccctattctcagtgtgccttcaacggcgtgtttctgccacccctccacgggagtttcggtgccttttcagctttctactttgtgatggacttctttaagaaagtggctaagaattctgtcatcagtcaggagaagatgactgaaattaccaagaacttctgctctaaaagttgggaggaaaccaagacatcatatcctagcgtgaaggagaaatacctgagcgaatattgtttttccggagcctacatcctgtccctgctccaggggtataatttcacagactcctcttgggagcagatccacttcatgggcaagatcaaggatagcaacgcagggtggaccctgggttacatgctgaatctcacaaacatgatcccagccgaacagcccctgtcccctccactgcctcactccacctaa

SEQ ID NO: 19 - protein, 1009 aa, Artificial
  soluble CD73-CD39 fusion derived from homo sapiens
MPSSVSWGILLLAGLCCLVPVSLAEWELTILHTNDVHSRLEQTSEDSSKCVNASRCMGGVARLFTKVQQIRRAEPNVLLLDAGDQYQGTIWFTVYKGAEVAHFMNALRYDAMALGNHEFDNGVEGLIEPLLKEAKFPILSANIKAKGPLASQISGLYLPYKVLPVGDEVVGIVGYTSKETPFLSNPGTNLVFEDEITALQPEVDKLKTLNVNKIIALGHSGFEMDKLIAQKVRGVDVVVGGHSNTFLYTGNPPSKEVPAGKYPFIVTSDDGRKVPVVQAYAFGKYLGYLKIEFDERGNVISSHGNPILLNSSIPEDPSIKADINKWRIKLDNYSTQELGKTIVYLDGSSQSCRFRECNMGNLICDAMINNNLRHADETFWNHVSMCILNGGGIRSPIDERNNGTITWENLAAVLPFGGTFDLVQLKGSTLKKAFEHSVHRYGQSTGEFLQVGGIHVVYDLSRKPGDRVVKLDVLCTKCRVPSYDPLKMDEVYKVILPNFLANGGDGFQMIKDELLRHDSGDQDINVVSTYISKMKVIYPAVEGRIKFASGGGAGGGAGGGAGGGAGGGTGTQNKALPENVKYGIVLDAGSSHTSLYIYKWPAEKENDTGVVHQVEECRVKGPGISKFVQKVNEIGIYLTDCMERAREVIPRSQHQETPVYLGATAGMRLLRMESEELADRVLDVVERSLSNYPFDFQGARIITGQEEGAYGWITINYLLGKFSQKTRWFSIVPYETNNQETFGALDLGGASTQVTFVPQNQTIESPDNALQFRLYGKDYNVYTHSFLCYGKDQALWQKLAKDIQVASNEILRDPCFHPGYKKVVNVSDLYKTPCTKRFEMTLPFQQFEIQGIGNYQQCHQSILELFNTSYCPYSQCAFNGIFLPPLQGDFGAFSAFYFVMKFLNLTSEKVSQEKVTEMMKKFCAQPWEEIKTSYAGVKEKYLSEYCFSGTYILSLLLQGYHFTADSWEHIHFIGKIQGSDAGWTLGYMLNLTNMIPAEQPLSTPLSHST

SEQ ID NO: 20 - DNA, 3030 bp, Artificial
  soluble CD73-CD39 fusion derived from homo sapiens, codon optimized
atgcccagcagcgtgagctggggcatcctgctgctggccggcctgtgctgcctggtgcccgtgagcctggccgagtgggagctgaccatcctgcacaccaacgacgtgcacagcagactggagcagaccagcgaggacagcagcaagtgcgtgaacgccagcagatgcatgggcggcgtggccagactgttcaccaaggtgcagcagatcagaagagccgagcccaacgtgctgctgctggacgccggcgaccagtaccagggcaccatctggttcaccgtgtacaagggcgccgaggtggcccacttcatgaacgccctgagatacgacgccatggccctgggcaaccacgagttcgacaacggcgtggagggcctgatcgagcccctgctgaaggaggccaagttccccatcctgagcgccaacatcaaggccaagggccccctggccagccagatcagcggcctgtacctgccctacaaggtgctgcccgtgggcgacgaggtggtgggcatcgtgggctacaccagcaaggagacccccttcctgagcaaccccggcaccaacctggtgttcgaggacgagatcaccgccctgcagcccgaggtggacaagctgaagaccctgaacgtgaacaagatcatcgccctgggccacagcggcttcgagatggacaagctgatcgcccagaaggtgagaggcgtggacgtggtggtgggcggccacagcaacaccttcctgtacaccggcaacccccccagcaaggaggtgcccgccggcaagtaccccttcatcgtgaccagcgacgacggcagaaaggtgcccgtggtgcaggcctacgccttcggcaagtacctgggctacctgaagatcgagttcgacgagagaggcaacgtgatcagcagccacggcaaccccatcctgctgaacagcagcatccccgaggaccccagcatcaaggccgacatcaacaagtggagaatcaagctggacaactacagcacccaggagctgggcaagaccatcgtgtacctggacggcagcagccagagctgcagattcagagagtgcaacatgggcaacctgatctgcgacgccatgatcaacaacaacctgagacacgccgacgagaccttctggaaccacgtgagcatgtgcatcctgaacggcggcggcatcagaagccccatcgacgagagaaacaacggcaccatcacctgggagaacctggccgccgtgctgcccttcggcggcaccttcgacctggtgcagctgaagggcagcaccctgaagaaggccttcgagcacagcgtgcacagatacggccagagcaccggcgagttcctgcaggtgggcggcatccacgtggtgtacgacctgagcagaaagcccggcgacagagtggtgaagctggacgtgctgtgcaccaagtgcagagtgcccagctacgaccccctgaagatggacgaggtgtacaaggtgatcctgcccaacttcctggccaacggcggcgacggcttccagatgatcaaggacgagctgctgagacacgacagcggcgaccaggacatcaacgtggtgagcacctacatcagcaagatgaaggtgatctaccccgccgtggagggcagaatcaagttcgccagcggcggcggcgccggcggcggcgccggcggcggcgccggcggcggcgccggcggcggcaccggcacccagaacaaggccctgcccgagaacgtgaagtacggcatcgtgctggacgccggcagcagccacaccagcctgtacatctacaagtggcccgccgagaaggagaacgacaccggcgtggtgcaccaggtggaggagtgcagagtgaagggccccggcatcagcaagttcgtgcagaaggtgaacgagatcggcatctacctgaccgactgcatggagagagccagagaggtgatccccagaagccagcaccaggagacccccgtgtacctgggcgccaccgccggcatgagactgctgagaatggagagcgaggagctggccgacagagtgctggacgtggtggagagaagcctgagcaactaccccttcgacttccagggcgccagaatcatcaccggccaggaggagggcgcctacggctggatcaccatcaactacctgctgggcaagttcagccagaagaccagatggttcagcatcgtgccctacgagaccaacaaccaggagaccttcggcgccctggacctgggcggcgccagcacccaggtgaccttcgtgccccagaaccagaccatcgagagccccgacaacgccctgcagttcagactgtacggcaaggactacaacgtgtacacccacagcttcctgtgctacggcaaggaccaggccctgtggcagaagctggccaaggacatccaggtggccagcaacgagatcctgagagacccctgcttccaccccggctacaagaaggtggtgaacgtgagcgacctgtacaagaccccctgcaccaagagattcgagatgaccctgcccttccagcagttcgagatccagggcatcggcaactaccagcagtgccaccagagcatcctggagctgttcaacaccagctactgcccctacagccagtgcgccttcaacggcatcttcctgccccccctgcagggcgacttcggcgccttcagcgccttctacttcgtgatgaagttcctgaacctgaccagcgagaaggtgagccaggagaaggtgaccgagatgatgaagaagttctgcgcccagccctgggaggagatcaagaccagctacgccggcgtgaaggagaagtacctgagcgagtactgcttcagcggcacctacatcctgagcctgctgctgcagggctaccacttcaccgccgacagctgggagcacatccacttcatcggcaagatccagggcagcgacgccggctggaccctgggctacatgctgaacctgaccaacatgatccccgccgagcagcccctgagcacccccctgagccacagcacctga

SEQ ID NO: 21 - protein, 21 aa, Artificial
  linker
ASGGGAGGGAGGGAGGGAGGG

SEQ ID NO: 22 - protein, 24 aa, Artificial
  hAAT signal sequence
MPSSVSWGILLLAGLCCLVPVSLA

SEQ ID NO: 23 - DNA, 166 bp, Artificial
  promoter
ctagcaggcctcgaggggactttccacaaggggactttccgtcgaggggactttccacaaggggactttccgtcgaggggactttccacaaggggactttccgtcgaggcctgtaggcgtgtacggtgggaggcttatataagcagagctcaagcttggtaccgag

SEQ ID NO: 24 - DNA, 130 bp, Artificial
  single stranded AAV2 ITR, 5' ITR
cctgcaggcagctgcgcgctcgctcgctcactgaggccgcccgggcgtcgggcgacctttggtcgcccggcctcagtgagcgagcgagcgcgcagagagggagtggccaactccatcactaggggttcct

SEQ ID NO: 25 - DNA, 142 bp, Artificial
  single stranded AAV2 ITR, 3'ITR
aggaacccctagtgatggagttggccactccctctctgcgcgctcgctcgctcactgaggccgggcgaccaaaggtcgcccgacgcccgggctttgcccgggcggcctcagtgagcgagcgagcgcgcagctgcctgcaggg

SEQ ID NO: 26 - DNA, 95 bp, Artificial
  double stranded AAV2 ITR, 5'ITR
ctgcgcgctcgctcgctcactgaggccgcccgggcgtcgggcgacctttggtcgcccggcctcagtgagcgagcgagcgcgcagagagggagtgg

SEQ ID NO: 27 - DNA, 142 bp, Artificial; identical to SEQ ID NO: 25
  double stranded AAV2 ITR, 3' ITR

SEQ ID NO: 28 - DNA, 167 bp, Artificial
  AAV5 ITR: 5'ITR
ctctcccccctgtcgcgttcgctcgctcgctggctcgtttgggggggtggcagctcaaagagctgccagacgacggccctctggccgtcgcccccccaaacgagccagcgagcgagcgaacgcgacaggggggagagtgccacactctcaagcaagggggttttgta

SEQ ID NO: 29 - DNA, 167 bp, Artificial
  AAV5 ITR: 3'ITR
tacaaaacctccttgcttgagagtgtggcactctcccccctgtcgcgttcgctcgctcgctggctcgtttgggggggtggcagctcaaagagctgccagacgacggccctctggccgtcgcccccccaaacgagccagcgagcgagcgaacgcgacaggggggagag

SEQ ID NO: 30 - DNA, 2208 bp, Artificial
  AAV2 Capsid
atggctgccgatggttatcttccagattggctcgaggacactctctctgaaggaataagacagtggtggaagctcaaacctggcccaccaccaccaaagcccgcagagcggcataaggacgacagcaggggtcttgtgcttcctgggtacaagtacctcggacccttcaacggactcgacaagggagagccggtcaacgaggcagacgccgcggccctcgagcacgacaaagcctacgaccggcagctcgacagcggagacaacccgtacctcaagtacaaccacgccgacgcggagtttcaggagcgccttaaagaagatacgtcttttgggggcaacctcggacgagcagtcttccaggcgaaaaagagggttcttgaacctctgggcctggttgaggaacctgttaagacggctccgggaaaaaagaggccggtagagcactctcctgtggagccagactcctcctcgggaaccggaaaggcgggccagcagcctgcaagaaaaagattgaattttggtcagactggagacgcagactcagtacctgacccccagcctctcggacagccaccagcagccccctctggtctgggaactaatacgatggctacaggcagtggcgcaccaatggcagacaataacgagggcgccgacggagtgggtaattcctcgggaaattggcattgcgattccacatggatgggcgacagagtcatcaccaccagcacccgaacctgggccctgcccacctacaacaaccacctctacaaacaaatttccagccaatcaggagcctcgaacgacaatcactactttggctacagcaccccttgggggtattttgacttcaacagattccactgccacttttcaccacgtgactggcaaagactcatcaacaacaactggggattccgacccaagagactcaacttcaagctctttaacattcaagtcaaagaggtcacgcagaatgacggtacgacgacgattgccaataaccttaccagcacggttcaggtgtttactgactcggagtaccagctcccgtacgtcctcggctcggcgcatcaaggatgcctcccgccgttcccagcagacgtcttcatggtgccacagtatggatacctcaccctgaacaacgggagtcaggcagtaggacgctcttcattttactgcctggagtactttccttctcagatgctgcgtaccggaaacaactttaccttcagctacacttttgaggacgttcctttccacagcagctacgctcacagccagagtctggaccgtctcatgaatcctctcatcgaccagtacctgtattacttgagcagaacaaacactccaagtggaaccaccacgcagtcaaggcttcagttttctcaggccggagcgagtgacattcgggaccagtctaggaactggcttcctggaccctgttaccgccagcagcgagtatcaaagacatctgcggataacaacaacagtgaatactcgtggactggagctaccaagtaccacctcaatggcagagactctctggtgaatccgggcccggccatggcaagccacaaggacgatgaagaaaagttttttcctcagagcggggttctcatctttgggaagcaaggctcagagaaaacaaatgtggacattgaaaaggtcatgattacagacgaagaggaaatcaggacaaccaatcccgtggctacggagcagtatggttctgtatctaccaacctccagagaggcaacagacaagcagctaccgcagatgtcaacacacaaggcgttcttccaggcatggtctggcaggacagagatgtgtaccttcaggggcccatctgggcaaagattccacacacggacggacattttcacccctctcccctcatgggtggattcggacttaaacaccctcctccacagattctcatcaagaacaccccggtacctgcgaatccttcgaccaccttcagtgcggcaaagtttgcttccttcatcacacagtactccacgggacaggtcagcgtggagatcgagtgggagctgcagaaggaaaacagcaaacgctggaatcccgaaattcagtacacttccaactacaacaagtctgttaatgtggactttactgtggacactaatggcgtgtattcagagcctcgccccattggcaccagatacctgactcgtaatctgtaa

SEQ ID NO: 31 - protein, 735 aa, Artificial [sequence omitted]

SEQ ID NO: 32 - protein, 598 aa, Artificial
  AAV2 VP2
TAPGKKRPVEHSPVEPDSSSGTGKAGQQPARKRLNFGQTGDADSVPDPQPLGQPPAAPSGLGTNTMATGSGAPMADNNEGADGVGNSSGNWHCDSTWMGDRVITTSTRTWALPTYNNHLYKQISSQSGASNDNHYFGYSTPWGYFDFNRFHCHFSPRDWQRLINNNWGFRPKRLNFKLFNIQVKEVTQNDGTTTIANNLTSTVQVFTDSEYQLPYVLGSAHQGCLPPFPADVFMVPQYGYLTLNNGSQAVGRSSFYCLEYFPSQMLRTGNNFTFSYTFEDVPFHSSYAHSQSLDRLMNPLIDQYLYYLSRTNTPSGTTTQSRLQFSQAGASDIRDQSRNWLPGPCYRQQRVSKTSADNNNSEYSWTGATKYHLNGRDSLVNPGPAMASHKDDEEKFFPQSGVLIFGKQGSEKTNVDIEKVMITDEEEIRTTNPVATEQYGSVSTNLQRGNRQAATADVNTQGVLPGMVWQDRDVYLQGPIWAKIPHTDGHFHPSPLMGGFGLKHPPPQILIKNTPVPANPSTTFSAAKFASFITQYSTGQVSVEIEWELQKENSKRWNPEIQYTSNYNKSVNVDFTVDTNGVYSEPRPIGTRYLTRNL

SEQ ID NO: 33 - protein, 533 aa, Artificial
  AAV2 VP3
MATGSGAPMADNNEGADGVGNSSGNWHCDSTWMGDRVITTSTRTWALPTYNNHLYKQISSQSGASNDNHYFGYSTPWGYFDFNRFHCHFSPRDWQRLINNNWGFRPKRLNFKLFNIQVKEVTQNDGTTTIANNLTSTVQVFTDSEYQLPYVLGSAHQGCLPPFPADVFMVPQYGYLTLNNGSQAVGRSSFYCLEYFPSQMLRTGNNFTFSYTFEDVPFHSSYAHSQSLDRLMNPLIDQYLYYLSRTNTPSGTTTQSRLQFSQAGASDIRDQSRNWLPGPCYRQQRVSKTSADNNNSEYSWTGATKYHLNGRDSLVNPGPAMASHKDDEEKFFPQSGVLIFGKQGSEKTNVDIEKVMITDEEEIRTTNPVATEQYGSVSTNLQRGNRQAATADVNTQGVLPGMVWQDRDVYLQGPIWAKIPHTDGHFHPSPLMGGFGLKHPPPQILIKNTPVPANPSTTFSAAKFASFITQYSTGQVSVEIEWELQKENSKRWNPEIQYTSNYNKSVNVDFTVDTNGVYSEPRPIGTRYLTRNL

SEQ ID NO: 34 - DNA, 2190 bp, Artificial
  AAV5 capsid
atgtcttttgttgatcaccctccagattggttggaagaagttggtgaaggtcttcgcgagtttttgggccttgaagcgggcccaccgaaaccaaaacccaatcagcagcatcaagatcaagcccgtggtcttgtgctgcctggttataactatctcggacccggaaacggtctcgatcgaggagagcctgtcaacagggcagacgaggtcgcgcgagagcacgacatctcgtacaacgagcagcttgaggcgggagacaacccctacctcaagtacaaccacgcggacgccgagtttcaggagaagctcgccgacgacacatccttcgggggaaacctcggaaaggcagtctttcaggccaagaaaagggttctcgaaccttttggcctggttgaagagggtgctaagacgtttaaacgcgatcgcgcccctaccggaaagcggatagacgaccactttccaaaaagaaagaaggctcggaccgaagaggactccaagccttccacctcgtcagacgccgaagctggacccagcggatcccagcagctgcaaatcccagcccaaccagcctcaagtttgggagctgatacaatgtctgcgggaggtggcggcccattgggcgacaataaccaaggtgccgatggagtgggcaatgcctcgggagattggcattgcgattccacgtggatgggggacagagtcgtcaccaagtccacccgaacctgggtgctgcccagctacaacaaccaccagtaccgagagatcaaaagcggctccgtcgacggaagcaacgccaacgcctactttggatacagcaccccctgggggtactttgactttaaccgcttccacagccactggagcccccgagactggcaaagactcatcaacaactactggggcttcagaccccggtccctcagagtcaaaatcttcaacattcaagtcaaagaggtcacggtgcaggactccaccaccaccatcgccaacaacctcacctccaccgtccaagtgtttacggacgacgactaccagctgccctacgtcgtcggcaacgggaccgagggatgcctgccggccttccctccgcaggtctttacgctgccgcagtacggttacgcgacgctgaaccgcgacaacacagaaaatcccaccgagaggagcagcttcttctgcctagagtactttcccagcaagatgctgagaacgggcaacaactttgagtttacctacaactttgaggaggtgcccttccactccagcttcgctcccagtcagaacctcttcaagctggccaacccgctggtggaccagtacttgtaccgcttcgtgagcacaaataacactggcggagtccagttcaacaagaacctggccgggagatacgccaacacctacaaaaactggttcccggggcccatgggccgaacccagggctggaacctgggctccggggtcaaccgcgccagtgtcagcgccttcgccacgaccaataggatggagctcgagggcgcgagttaccaggtgcccccgcagccgaacggcatgaccaacaacctccagggcagcaacacctatgccctggagaacactatgatcttcaacagccagccggcgaacccgggcaccaccgccacgtacctcgagggcaacatgctcatcaccagcgagagcgagacgcagccggtgaaccgcgtggcgtacaacgtcggcgggcagatggccaccaacaaccagagctccaccactgcccccgcgaccggcacgtacaacctccaggaaatcgtgcccggcagcgtgtggatggagagggacgtgtacctccaaggacccatctgggccaagatcccagagacgggggcgcactttcacccctctccggccatgggcggattcggactcaaacacccaccgcccatgatgctcatcaagaacacgcctgtgcccggaaatatcaccagcttctcggacgtgcccgtcagcagcttcatcacccagtacagcaccgggcaggtcaccgtggagatggagtgggagctcaagaaggaaaactccaagaggtggaacccagagatccagtacacaaacaactacaacgacccccagtttgtggactttgccccggacagcaccggggaatacagaaccaccagacctatcggaacccgataccttacccgacccctttaa

SEQ ID NO: 35 - protein, 729 aa, Artificial
  AAV5 VP1
MSFVDHPPDWLEEVGEGLREFLGLEAGPPKPKPNQQHQDQARGLVLPGYNYLGPGNGLDRGEPVNRADEVAREHDISYNEQLEAGDNPYLKYNHADAEFQEKLADDTSFGGNLGKAVFQAKKRVLEPFGLVEEGAKTFKRDRAPTGKRIDDHFPKRKKARTEEDSKPSTSSDAEAGPSGSQQLQIPAQPASSLGADTMSAGGGGPLGDNNQGADGVGNASGDWHCDSTWMGDRVVTKSTRTWVLPSYNNHQYREIKSGSVDGSNANAYFGYSTPWGYFDFNRFHSHWSPRDWQRLINNYWGFRPRSLRVKIFNIQVKEVTVQDSTTTIANNLTSTVQVFTDDDYQLPYVVGNGTEGCLPAFPPQVFTLPQYGYATLNRDNTENPTERSSFFCLEYFPSKMLRTGNNFEFTYNFEEVPFHSSFAPSQNLFKLANPLVDQYLYRFVSTNNTGGVQFNKNLAGRYANTYKNWFPGPMGRTQGWNLGSGVNRASVSAFATTNRMELEGASYQVPPQPNGMTNNLQGSNTYALENTMIFNSQPANPGTTATYLEGNMLITSESETQPVNRVAYNVGGQMATNNQSSTTAPATGTYNLQEIVPGSVWMERDVYLQGPIWAKIPETGAHFHPSPAMGGFGLKHPPPMMLIKNTPVPGNITSFSDVPVSSFITQYSTGQVTVEMEWELKKENSKRWNPEIQYTNNYNDPQFVDFAPDSTGEYRTTRPIGTRYLTRPL

SEQ ID NO: 36 - protein, 593 aa, Artificial
  AAV5 VP2
TFKRDRAPTGKRIDDHFPKRKKARTEEDSKPSTSSDAEAGPSGSQQLQIPAQPASSLGADTMSAGGGGPLGDNNQGADGVGNASGDWHCDSTWMGDRVVTKSTRTWVLPSYNNHQYREIKSGSVDGSNANAYFGYSTPWGYFDFNRFHSHWSPRDWQRLINNYWGFRPRSLRVKIFNIQVKEVTVQDSTTTIANNLTSTVQVFTDDDYQLPYVVGNGTEGCLPAFPPQVFTLPQYGYATLNRDNTENPTERSSFFCLEYFPSKMLRTGNNFEFTYNFEEVPFHSSFAPSQNLFKLANPLVDQYLYRFVSTNNTGGVQFNKNLAGRYANTYKNWFPGPMGRTQGWNLGSGVNRASVSAFATTNRMELEGASYQVPPQPNGMTNNLQGSNTYALENTMIFNSQPANPGTTATYLEGNMLITSESETQPVNRVAYNVGGQMATNNQSSTTAPATGTYNLQEIVPGSVWMERDVYLQGPIWAKIPETGAHFHPSPAMGGFGLKHPPPMMLIKNTPVPGNITSFSDVPVSSFITQYSTGQVTVEMEWELKKENSKRWNPEIQYTNNYNDPQFVDFAPDSTGEYRTTRPIGTRYLTRPL

SEQ ID NO: 37 - protein, 532 aa, Artificial
  AAV5 VP3
MSAGGGGPLGDNNQGADGVGNASGDWHCDSTWMGDRVVTKSTRTWVLPSYNNHQYREIKSGSVDGSNANAYFGYSTPWGYFDFNRFHSHWSPRDWQRLINNYWGFRPRSLRVKIFNIQVKEVTVQDSTTTIANNLTSTVQVFTDDDYQLPYVVGNGTEGCLPAFPPQVFTLPQYGYATLNRDNTENPTERSSFFCLEYFPSKMLRTGNNFEFTYNFEEVPFHSSFAPSQNLFKLANPLVDQYLYRFVSTNNTGGVQFNKNLAGRYANTYKNWFPGPMGRTQGWNLGSGVNRASVSAFATTNRMELEGASYQVPPQPNGMTNNLQGSNTYALENTMIFNSQPANPGTTATYLEGNMLITSESETQPVNRVAYNVGGQMATNNQSSTTAPATGTYNLQEIVPGSVWMERDVYLQGPIWAKIPETGAHFHPSPAMGGFGLKHPPPMMLIKNTPVPGNITSFSDVPVSSFITQYSTGQVTVEMEWELKKENSKRWNPEIQYTNNYNDPQFVDFAPDSTGEYRTTRPIGTRYLTRPL

SEQ ID NO: 38 - DNA, 2217 bp, Artificial
  AAV8 capsid
atggctgccgatggttatcttccagattggctcgaggacaacctctctgagggcattcgcgagtggtgggcgctgaaacctggagccccgaagcccaaagccaaccagcaaaagcaggacgacggccggggtctggtgcttcctggctacaagtacctcggacccttcaacggactcgacaagggggagcccgtcaacgcggcggacgcagcggccctcgagcacgacaaggcctacgaccagcagctgcaggcgggtgacaatccgtacctgcggtataaccacgccgacgccgagtttcaggagcgtctgcaagaagatacgtcttttgggggcaacctcgggcgagcagtcttccaggccaagaagcgggttctcgaacctctcggtctggttgaggaaggcgctaagacggctcctggaaagaagagaccggtagagccatcaccccagcgttctccagactcctctacgggcatcggcaagaaaggccaacagcccgccagaaaaagactcaattttggtcagactggcgactcagagtcagttccagaccctcaacctctcggagaacctccagcagcgccctctggtgtgggacctaatacaatggctgcaggcggtggcgcaccaatggcagacaataacgaaggcgccgacggagtgggtagttcctcgggaaattggcattgcgattccacatggctgggcgacagagtcatcaccaccagcacccgaacctgggccctgcccacctacaacaaccacctctacaagcaaatctccaacgggacatcgggaggagccaccaacgacaacacctacttcggctacagcaccccctgggggtattttgactttaacagattccactgccacttttcaccacgtgactggcagcgactcatcaacaacaactggggattccggcccaagagactcagcttcaagctcttcaacatccaggtcaaggaggtcacgcagaatgaaggcaccaagaccatcgccaataacctcaccagcaccatccaggtgtttacggactcggagtaccagctgccgtacgttctcggctctgcccaccagggctgcctgcctccgttcccggcggacgtgttcatgattccccagtacggctacctaacactcaacaacggtagtcaggccgtgggacgctcctccttctactgcctggaatactttccttcgcagatgctgagaaccggcaacaacttccagtttacttacaccttcgaggacgtgcctttccacagcagctacgcccacagccagagcttggaccggctgatgaatcctctgattgaccagtacctgtactacttgtctcggactcaaacaacaggaggcacggcaaatacgcagactctgggcttcagccaaggtgggcctaatacaatggccaatcaggcaaagaactggctgccaggaccctgttaccgccaacaacgcgtctcaacgacaaccgggcaaaacaacaatagcaactttgcctggactgctgggaccaaataccatctgaatggaagaaattcattggctaatcctggcatcgctatggcaacacacaaagacgacgaggagcgtttttttcccagtaacgggatcctgatttttggcaaacaaaatgctgccagagacaatgcggattacagcgatgtcatgctcaccagcgaggaagaaatcaaaaccactaaccctgtggctacagaggaatacggtatcgtggcagataacttgcagcagcaaaacacggctcctcaaattggaactgtcaacagccagggggccttacccggtatggtctggcagaaccgggacgtgtacctgcagggtcccatctgggccaagattcctcacacggacggcaacttccacccgtctccgctgatgggcggctttggcctgaaacatcctccgcctcagatcctgatcaagaacacgcctgtacctgcggatcctccgaccaccttcaaccagtcaaagctgaactctttcatcacgcaatacagcaccggacaggtcagcgtggaaattgaatgggagctgcagaaggaaaacagcaagcgctggaaccccgagatccagtacacctccaactactacaaatctacaagtgtggactttgctgttaatacagaaggcgtgtactctgaaccccgccccattggcacccgttacctcacccgtaatctgtaa

SEQ ID NO: 39 - protein, 782 aa, Artificial
  AAV8 VP1
MAADGYLPDWLEDNLSEGIREWWALKPGAPKPKANQQKQDDGRGLVLPGYKYLGPFNGLDKGEPVNAADAAALEHDKAYDQQLQAGDNPYLRYNHADAEFQERLQEDTSFGGNLGRAVFQAKKRVLEPLGLVEEGAKTAPGKKRPVEPSPQRSPDSSTGIGKKGQQPARKRLNFGQTGDSESVPDPQPLGEPPAAPSGVGPNTMAAGGGAPMADNNEGADGVGSSSGNWHCDSTWLGDRVITTSTRTWALPTYNNHLYKQISNGTSGGATNDNTYFGYSTPWGYFDFNRFHCHFSPRDWQRLINNNWGFRPKRLSFKLFNIQVKEVTQNEGTKTIANNLTSTIQVFTDSEYQLPYVLGSAHQGCLPPFPADVFMIPQYGYLTLNNGSQAVGRSSFYCLEYFPSQMLRTGNNFQFTYTFEDVPFHSSYAHSQSLDRLMNPLIDQYLYYLSRTQTTGGTANTQTLGFSQGGPNTMANQAKNWLPGPCYRQQRVSTTTGQNNNSNFAWTAGTKYHLNGRNSLANPGIAMATHKDDEERFFPSNGILIFGKQNAARDNADYSDVMLTSEEEIKTTNPVATEEYGIVADNLQQQNTAPQIGTVNSQGALPGMVWQNRDVYLQGPIWAKIPHTDGNFHPSPLMGGFGLKHPPPQILIKNTPVPADPPTTFNQSKLNSFITQYSTGQVSVEIEWELQKENSKRWNPEIQYTSNYYKSTSVDFAVNTEGVYSEPRPIGTRYLTRNLMAADGYLPDWLEDNLSEGIREWWALKPGAPKPKANQQKQDDGRG

SEQ ID NO: 40 - protein, 601 aa, Artificial
  AAV8 VP2
TAPGKKRPVEPSPQRSPDSSTGIGKKGQQPARKRLNFGQTGDSESVPDPQPLGEPPAAPSGVGPNTMAAGGGAPMADNNEGADGVGSSSGNWHCDSTWLGDRVITTSTRTWALPTYNNHLYKQISNGTSGGATNDNTYFGYSTPWGYFDFNRFHCHFSPRDWQRLINNNWGFRPKRLSFKLFNIQVKEVTQNEGTKTIANNLTSTIQVFTDSEYQLPYVLGSAHQGCLPPFPADVFMIPQYGYLTLNNGSQAVGRSSFYCLEYFPSQMLRTGNNFQFTYTFEDVPFHSSYAHSQSLDRLMNPLIDQYLYYLSRTQTTGGTANTQTLGFSQGGPNTMANQAKNWLPGPCYRQQRVSTTTGQNNNSNFAWTAGTKYHLNGRNSLANPGIAMATHKDDEERFFPSNGILIFGKQNAARDNADYSDVMLTSEEEIKTTNPVATEEYGIVADNLQQQNTAPQIGTVNSQGALPGMVWQNRDVYLQGPIWAKIPHTDGNFHPSPLMGGFGLKHPPPQILIKNTPVPADPPTTFNQSKLNSFITQYSTGQVSVEIEWELQKENSKRWNPEIQYTSNYYKSTSVDFAVNTEGVYSEPRPIGTRYLTRNL

SEQ ID NO: 41 - protein, 535 aa, Artificial
  AAV8 VP3
MAAGGGAPMADNNEGADGVGSSSGNWHCDSTWLGDRVITTSTRTWALPTYNNHLYKQISNGTSGGATNDNTYFGYSTPWGYFDFNRFHCHFSPRDWQRLINNNWGFRPKRLSFKLFNIQVKEVTQNEGTKTIANNLTSTIQVFTDSEYQLPYVLGSAHQGCLPPFPADVFMIPQYGYLTLNNGSQAVGRSSFYCLEYFPSQMLRTGNNFQFTYTFEDVPFHSSYAHSQSLDRLMNPLIDQYLYYLSRTQTTGGTANTQTLGFSQGGPNTMANQAKNWLPGPCYRQQRVSTTTGQNNNSNFAWTAGTKYHLNGRNSLANPGIAMATHKDDEERFFPSNGILIFGKQNAARDNADYSDVMLTSEEEIKTTNPVATEEYGIVADNLQQQNTAPQIGTVNSQGALPGMVWQNRDVYLQGPIWAKIPHTDGNFHPSPLMGGFGLKHPPPQILIKNTPVPADPPTTFNQSKLNSFITQYSTGQVSVEIEWELQKENSKRWNPEIQYTSNYYKSTSVDFAVNTEGVYSEPRPIGTRYLTRNL

SEQ ID NO: 42 - DNA, 7494 bp, Artificial
  pAAV-CMV-CD39-2A-CD73
cctgcaggcagctgcgcgctcgctcgctcactgaggccgcccgggcaaagcccgggcgtcgggcgacctttggtcgcccggcctcagtgagcgagcgagcgcgcagagagggagtggccaactccatcactaggggttcctgcggccgcacgcgtcgacattgattattgactagttattaatagtaatcaattacggggtcattagttcatagcccatatatggagttccgcgttacataacttacggtaaatggcccgcctggctgaccgcccaacgacccccgcccattgacgtcaataatgacgtatgttcccatagtaacgccaatagggactttccattgacgtcaatgggtggactatttacggtaaactgcccacttggcagtacatcaagtgtatcatatgccaagtacgccccctattgacgtcaatgacggtaaatggcccgcctggcattatgcccagtacatgaccttatgggactttcctacttggcagtacatctacgtattagtcatcgctattaccatggtgatgcggttttggcagtacatcaatgggcgtggatagcggtttgactcacggggatttccaagtctccaccccattgacgtcaatgggagtttgttttggcaccaaaatcaacgggactttccaaaatgtcgtaacaactccgccccattgacgcaaatgggcggtaggcgtgtacggtgggaggtctatataagcagagctctctggctaactagagaacccactgcttactggcttatcgaaattaatacgactcactatagggagacccaagctggctagttaagcttggtaccgagctcggatcgccaccatgagccgcatggaggacatcaaagactcaaaagtgaaaagattctgctcaaaaaacattctcatcattctggggtttacatcaattctcgctgtgatcgcactgattgccgtcggcctcactcagaacaagcccctgcctgagaacgtgaagtacggaatcgtcctggacgctgggagctcccacaccaatctgtacatctacaagtggccagcagagaaagaaaacgatacaggcgtggtccagcagctggaggaatgccaggtgaagggtcccggcatctccaagtacgcccagaaaacagacgagattggagcttatctggcagagtgtatggaactgagcacagaactcatccccacttccaagcaccatcagacacccgtgtacctgggtgcaactgcaggaatgcgactgctccgcatggagtcagaacagagcgccgacgaggtgctggcagctgtcagtacttcactcaaatcttatccattcgattttcagggtgccaagatcattaccggccaggaggaaggagcttacgggtggatcactattaactatctgctcgggcggttcacccaggagcagtcctggctgtctctcatcagcgactcccagaagcaggaaaccttcggcgctctggatctcggcggagcaagcacccagatcacatttgtgccacagaatagcacaattgagtcccccgaaaactctctgcagttccgcctctacggggaggactacaccgtgtacacccactcctttctgtgctatggcaaggaccaggccctgtggcagaagctcgctaaagatatccaggtgtctagtgggggtgtcctgaaagatccctgcttcaatcctggttacgagaaggtggtcaacgtgtctgaactgtatggaacaccatgtactaagaggttcgagaagaaactgcccttcgaccagtttcgaatccagggaaccggggattacgagcagtgtcaccagagcattctggaactcttcaacaatagccattgcccatattcccagtgtgccttcaacggagtgtttctgccccctctccacggttctttcggcgcctttagtgctttctactttgtgatggacttctttaagaaagtggctaagaatagtgtcatctcacaggagaagatgaccgaaatcacaaagaacttctgctctaagagttgggaggaaaccaagacaagctacccctccgtgaaggagaaatacctgtcagaatattgttttagcggtgcctacatcctgtccctgctccagggctataatttcaccgactcaagctgggagcagatccactttatgggcaagatcaaggattctaacgccggatggaccctggggtacatgctgaatctcacaaacatgatcccagctgagcagccactgtccccaccactccctcattctacctatattggcctgatggtgctcttctccctgctcctggtggctgtcgcaatcacaggactgttcatctactctaagccaagttatttttggaaagaggcagtgggtagtggcgccacaaatttttcactcctgaagcaggccggagacgtggaggaaaacccagggcccatgaggcctgcagccgctaaggtgccaaaatggctcctgctcgcactgtccgccctgctccctcagtggccagcagcctctgcttgggagctgactatcctccacaccaatgatgtgcatagtagactggaacagacctcagacgatagcacaaagtgcctgaacgccagcctgtgcgtgggaggagtcgcaagactgttcaccaaggtgcagcagatccggaaagaggaacctaatgtcctgtttctcgacgcaggcgaccagtaccagggcacaatctggttcaccgtgtacaagggactggaggtcgctcactttatgaacattctgggttacgacgccatggctctcggcaatcatgagttcgacaacggagtggaagggctgatcgatcctctgctccggaatgtgaaatttccaatcctgtcagctaacattaaggcacgaggtcctctggcacaccagatcagcggactgttcctcccaagtaaagtgctgtcagtcgggggcgaggtggtcggtattgtgggctacacctctaaggaaacacccttcctgagtaatcctggcacaaacctcgtgtttgaggacgaaatctctgccctgcagcctgaggtggataagctgaaaactctcaatgtcaacaagatcattgcactgggacacagcgggttcgaaatggacaagctgatcgcccagaaagtgagaggggtcgatattgtggtcggcggacatagtaatactttcctgtacaccggaaaccctccatcaaaggaggtgccagctgggaaatatccctttatcgtgaccgcagacgatggccggcaggtcccagtggtccaggcatacgccttcggcaagtacctgggctatctcaaagtggagtttgacgataagggaaacgtcatcacaagctatgggaatcccatcctgctcaactcctctattcctgaagacgccactatcaaagctgatattaatcagtggaggatcaagctggacaactactccactcaggagctgggaagaaccatcgtgtacctggatgggtctactcagacctgcaggttcagagaatgtaatatgggcaacctgatctgcgacgccatgattaacaataacctgcgacaccccgatgagatgttttggaatcatgtgagcatgtgcatcgtcaacgggggtggcatcaggtcccccattgacgagaagaataacggaacaattacttgggaaaacctggctgcagtgctccctttcggagggacatttgatctggtccagctcaaggggtccactctgaagaaagccttcgagcactcagtgcatcgctacggacagagcaccggggaatttctgcaagtgggtggcatccacgtggtctatgacattaatcgaaaaccctggaacagggtggtccagctggaggtgctctgcactaagtgtcgagtccctatctacgagccactggaaatggacaaggtgtacaaagtcaccctgcctagctatctcgccaacggaggggatggattccagatgattaaggacgagctgctcaaacatgattctggggaccaggatatctccgtggtctctgagtacattagtaagatgaaagtggtctatcctgctgtggaaggcaggatcaagttcagtgccgcttcacattaccagggttcttttccactcgtgattctctctttttgggctatgattctgattctctaatatcagtgaggatccacttaagggcgaattccagcacactggcggccgttagatctacgggtggcatccctgtgacccctccccagtgcctctcctggccctggaagttgccactccagtgcccaccagccttgtcctaataaaattaagttgcatcattttgtctgactaggtgtccttctataatattatggggtggaggggggtggtatggagcaaggggcaagttgggaagacaacctgtagggcctgcggggtctattgggaaccaagctggagtgcagtggcacaatcttggctcactgcaatctccgcctcctgggttcaagcgattctcctgcctcagcctcccgagttgttgggattccaggcatgcatgaccaggctcagctaatttttgtttttttggtagagacggggtttcaccatattggccaggctggtctccaactcctaatctcaggtgatctacccaccttggcctcccaaattgctgggattacaggcgtgaaccactgctcccttccctgtccttctgattttgtaggtaaccacgtgcggaccgagcggccgcaggaacccctagtgatggagttggccactccctctctgcgcgctcgctcgctcactgaggccgggcgaccaaaggtcgcccgacgcccgggctttgcccgggcggcctcagtgagcgagcgagcgcgcagctgcctgcaggggcgcctgatgcggtattttctccttacgcatctgtgcggtatttcacaccgcatacgtcaaagcaaccatagtacgcgccctgtagcggcgcattaagcgcggcgggtgtggtggttacgcgcagcgtgaccgctacacttgccagcgccctagcgcccgctcctttcgctttcttcccttcctttctcgccacgttcgccggctttccccgtcaagctctaaatcgggggctccctttagggttccgatttagtgctttacggcacctcgaccccaaaaaacttgatttgggtgatggttcacgtagtgggccatcgccctgatagacggtttttcgccctttgacgttggagtccacgttctttaatagtggactcttgttccaaactggaacaacactcaaccctatctcgggctattcttttgatttataagggattttgccgatttcggcctattggttaaaaaatgagctgatttaacaaaaatttaacgcgaattttaacaaaatattaacgtttacaattttatggtgcactctcagtacaatctgctctgatgccgcatagttaagccagccccgacacccgccaacacccgctgacgcgccctgacgggcttgtctgctcccggcatccgcttacagacaagctgtgaccgtctccgggagctgcatgtgtcagaggttttcaccgtcatcaccgaaacgcgcgagacgaaagggcctcgtgatacgcctatttttataggttaatgtcatgataataatggtttcttagacgtcaggtggcacttttcggggaaatgtgcgcggaacccctatttgtttatttttctaaatacattcaaatatgtatccgctcatgagacaataaccctgataaatgcttcaataatattgaaaaaggaagagtatgagtattcaacatttccgtgtcgcccttattcccttttttgcggcattttgccttcctgtttttgctcacccagaaacgctggtgaaagtaaaagatgctgaagatcagttgggtgcacgagtgggttacatcgaactggatctcaacagcggtaagatccttgagagttttcgccccgaagaacgttttccaatgatgagcacttttaaagttctgctatgtggcgcggtattatcccgtattgacgccgggcaagagcaactcggtcgccgcatacactattctcagaatgacttggttgagtactcaccagtcacagaaaagcatcttacggatggcatgacagtaagagaattatgcagtgctgccataaccatgagtgataacactgcggccaacttacttctgacaacgatcggaggaccgaaggagctaaccgcttttttgcacaacatgggggatcatgtaactcgccttgatcgttgggaaccggagctgaatgaagccataccaaacgacgagcgtgacaccacgatgcctgtagcaatggcaacaacgttgcgcaaactattaactggcgaactacttactctagcttcccggcaacaattaatagactggatggaggcggataaagttgcaggaccacttctgcgctcggcccttccggctggctggtttattgctgataaatctggagccggtgagcgtgggtctcgcggtatcattgcagcactggggccagatggtaagccctcccgtatcgtagttatctacacgacggggagtcaggcaactatggatgaacgaaatagacagatcgctgagataggtgcctcactgattaagcattggtaactgtcagaccaagtttactcatatatactttagattgatttaaaacttcatttttaatttaaaaggatctaggtgaagatcctttttgataatctcatgaccaaaatcccttaacgtgagttttcgttccactgagcgtcagaccccgtagaaaagatcaaaggatcttcttgagatcctttttttctgcgcgtaatctgctgcttgcaaacaaaaaaaccaccgctaccagcggtggtttgtttgccggatcaagagctaccaactctttttccgaaggtaactggcttcagcagagcgcagataccaaatactgtccttctagtgtagccgtagttaggccaccacttcaagaactctgtagcaccgcctacatacctcgctctgctaatcctgttaccagtggctgctgccagtggcgataagtcgtgtcttaccgggttggactcaagacgatagttaccggataaggcgcagcggtcgggctgaacggggggttcgtgcacacagcccagcttggagcgaacgacctacaccgaactgagatacctacagcgtgagctatgagaaagcgccacgcttcccgaagggagaaaggcggacaggtatccggtaagcggcagggtcggaacaggagagcgcacgagggagcttccagggggaaacgcctggtatctttatagtcctgtcgggtttcgccacctctgacttgagcgtcgatttttgtgatgctcgtcaggggggcggagcctatggaaaaacgccagcaacgcggcctttttacggttcctggccttttgctggccttttgctcacatgt

SEQ ID NO: 43 - DNA, 30 bp, Artificial
  primer
gcgaagcttaccatgagccgcatggaggac

SEQ ID NO: 44 - DNA, 38 bp, Artificial
  primer
gcgagatctttatcacactgcctctttccaaaaataac

SEQ ID NO: 45 - DNA, 32 bp, Artificial
  primer
gcgaagcttaccatgaggcctgcagccgctaa

SEQ ID NO: 46 - DNA, 35 bp, Artificial
  primer
gcgagatctttatcagagaatcagaatcatagccc

SEQ ID NO: 47 - DNA, 36 bp, Artificial
  primer
gcgagatctttatcagaacttgatcctgccttccac

SEQ ID NO: 48 - DNA, 1419 bp, homo sapiens
atggccgggaaggtgcggtcactgctgccgccgctgctgctggccgccgcgggcctcgccggcctcctactgctgtgcgtccccacccgcgacgtccgggagccgcccgccctcaagtatggcatcgtcctggatgctggttcttcacacacgtccatgtttatctacaagtggccggcagacaaggagaacgacacaggcattgtgggccagcacagctcctgtgatgttccaggtgggggcatctccagctatgcagacaacccttctggggccagccagagtcttgttggatgcctcgaacaggcgcttcaggatgtgcccaaagagagacacgcgggcacacccctctacctgggagccacagcgggtatgcgcctgctcaacctgaccaatccagaggcctcgaccagtgtgctcatggcagtgactcacacactgacccagtacccctttgacttccggggtgcacgcatcctctcgggccaagaagaaggggtgtttggctgggtgactgccaactacctgctggagaacttcatcaagtacggctgggtgggccggtggttccggccacggaaggggacactgggggccatggacctggggggtgcctctacccagatcacttttgagacaaccagtccagctgaggacagagccagcgaggtccagctgcatctctacggccagcactaccgagtctacacccacagcttcctctgctatggccgtgaccaggtcctccagaggctgctggccagcgccctccagacccacggcttccacccctgctggccgaggggcttttccacccaagtgctgctcggggatgtgtaccagtcaccatgcaccatggcccagcggccccagaacttcaacagcagtgccagggtcagcctgtcagggagcagtgacccccacctctgccgagatctggtttctgggctcttcagcttctcctcctgccccttctcccgatgctctttcaatggggtcttccagcccccagtggctgggaactttgtggccttctctgccttcttctacactgtggactttttgcggacttcgatggggctgcccgtggccaccctgcagcagctggaggcagccgcagtgaatgtctgcaaccagacctgggctcagcagctgctgagtcgcggctacggcttcgatgagcgcgccttcggcggcgtgatcttccagaagaaggccgcggacactgcagtgggctgggcgctcggctacatgctgaacctgaccaacctgatccccgccgacccgccggggctgcgcaagggcacagacttcagctcctgggtcgtcctcctgctgctcttcgcctccgcgctcctggctgcgcttgtcctgctgctgcgtcaggtgcactccgccaagctgccaagcaccatttag

SEQ ID NO: 49 - protein, 472 aa, homo sapiens
MAGKVRSLLPPLLLAAAGLAGLLLLCVPTRDVREPPALKYGIVLDAGSSHTSMFIYKWPADKENDTGIVGQHSSCDVPGGGISSYADNPSGASQSLVGCLEQALQDVPKERHAGTPLYLGATAGMRLLNLTNPEASTSVLMAVTHTLTQYPFDFRGARILSGQEEGVFGWVTANYLLENFIKYGWVGRWFRPRKGTLGAMDLGGASTQITFETTSPAEDRASEVQLHLYGQHYRVYTHSFLCYGRDQVLQRLLASALQTHGFHPCWPRGFSTQVLLGDVYQSPCTMAQRPQNFNSSARVSLSGSSDPHLCRDLVSGLFSFSSCPFSRCSFNGVFQPPVAGNFVAFSAFFYTVDFLRTSMGLPVATLQQLEAAAVNVCNQTWAQQLLSRGYGFDERAFGGVIFQKKAADTAVGWALGYMLNLTNLIPADPPGLRKGTDFSSWVVLLLLFASALLAALVLLLRQVHSAKLPSTI

SEQ ID NO: 50 - DNA, 1488 bp, Homo sapiens
atggggctgtcccggaaggagcaggtcttcttggccctgctgggggcctcgggggtctcaggcctcacggcactcattctcctcctggtggaggccaccagcgtgctcctgcccacagacatcaagtttgggatcgtgtttgatgcgggctcctcccacacgtccctcttcctgtatcagtggctggcgaacaaggagaatggcacgggtgtggtcagccaggccctggcctgccaggtggaagggcctggaatctcctcctacacttctaatgctgcacaggctggtgagagcctgcagggctgcttggaggaggcgctggtgctgatcccagaggcccagcatcggaaaacacccacgttcctgggggccacggctggcatgaggttgctcagccggaagaacagctctcaggccagggacatctttgcagcagtcacccaggtcctgggccggtctcccgtggacttttggggtgccgagctcctggccgggcaggccgaaggtgcctttggttggatcactgtcaactacggcttggggacgctggtcaagtactccttcactggagaatggatccagcctccggaggagatgctggtgggtgccctggacatgggaggggcctccacccagatcacgttcgtgcctgggggccccatcttggacaagagcacccaggccgattttcgcctctacggctccgactacagcgtctacactcacagctacctgtgctttggacgggaccagatgctgagcaggctcctcgtggggctggtacagagccgcccggctgccctgctccgtcacccgtgctacctcagcggctaccagaccacactggccctgggcccgctgtatgagtcaccctgtgtccacgccacgcccccgctgagcctcccccagaacctcacagttgaagggacaggcaaccctggagcctgcgtctcagccatccgggaacttttcaacttctccagctgccagggccaggaggactgcgcctttgacggggtctaccagcccccgctgcggggccagttctatgccttctccaacttctactacaccttccacttcctgaacctcacctccaggcagcccctgagcacggtcaacgccaccatctgggagttttgccagaggccctggaaactggtggaggccagctaccctgggcaggaccgctggctgcgggactactgtgcctcaggcctgtacatcctcaccctcctgcacgagggctacgggttcagcgaggagacctggcccagcctcgagttccgaaagcaggcgggcggtgtggacattggctggacactgggctacatgctgaacctgaccgggatgatcccggccgatgcgccggctcagtggcgggcagagagctacggcgtctgggtggccaaagtggtgttcatggtgctggccctggtggcggtggtgggggctgccttggtccagctcttctggttgcaggactag

SEQ ID NO: 51 - protein, 495 aa, Homo sapiens
MGLSRKEQVFLALLGASGVSGLTALILLLVEATSVLLPTDIKFGIVFDAGSSHTSLFLYQWLANKENGTGVVSQALACQVEGPGISSYTSNAAQAGESLQGCLEEALVLIPEAQHRKTPTFLGATAGMRLLSRKNSSQARDIFAAVTQVLGRSPVDFWGAELLAGQAEGAFGWITVNYGLGTLVKYSFTGEWIQPPEEMLVGALDMGGASTQITFVPGGPILDKSTQADFRLYGSDYSVYTHSYLCFGRDQMLSRLLVGLVQSRPAALLRHPCYLSGYQTTLALGPLYESPCVHATPPLSLPQNLTVEGTGNPGACVSAIRELFNFSSCQGQEDCAFDGVYQPPLRGQFYAFSNFYYTFHFLNLTSRQPLSTVNATIWEFCQRPWKLVEASYPGQDRWLRDYCASGLYILTLLHEGYGFSEETWPSLEFRKQAGGVDIGWTLGYMLNLTGMIPADAPAQWRAESYGVWVAKVVFMVLALVAVVGAALVQLFWLQD

SEQ ID NO: 52 - DNA, 3822 bp, Artificial
  Fc-tagged CD73-39 fusion DNA derived from mus musculus
atgggctggtcctgcatcatcctgttcctggtcgcaaccgcaactggcgtccattcagataaaactcatacttgtccaccttgtcctgctcctgagctgctgggaggaccaagcgtgttcctgtttccccctaagccaaaagacaccctgatgatcagccggactcccgaagtcacctgcgtggtcgtggacgtgagccacgaggatcccgaagtcaagttcaactggtacgtggatggcgtcgaggtgcataatgccaagacaaaacctagggaggaacagtacaactccacctatcgcgtcgtgtctgtcctgacagtgctgcaccaggactggctgaacggcaaagagtataagtgcaaagtgtccaataaggccctgcccgctcctatcgagaaaactatttctaaggctaaagggcagccacgagaaccacaggtgtacaccctgccaccaagccgggaggaaatgacaaagaaccaggtcagtctgacttgtctggtgaaaggattctatcctagcgacattgcagtggagtgggaatccaatggccagccagaaaacaattacaagaccacacctccagtgctggactctgatgggagtttctttctgtatagtaagctgacagtggataaatcacggtggcagcagggaaacgtcttttcttgcagtgtgatgcatgaggcactgcacaatcattacactcagaagtcactgagcctgtcccccggcaaagccgctgcaaatagctccatcgacctgatttcagtccccgtggatagccggagacctgcctgtaagattcctaacgacctgaaacagaaagtgatgaaccacgactacaaagacgacgacgacaaagagtgggaactgacaatcctgcacaccaatgacgtgcatagtcggctcgagcagacatcagacgatagcactaagtgcctgaacgccagcctgtgcgtgggaggagtcgcaagactgttcacaaaggtgcagcagatccggaaagaggaacctaatgtcctgtttctcgacgctggcgatcagtaccagggaacaatctggttcaccgtgtacaagggcctggaggtcgcacactttatgaacattctggggtacgacgctatggcactcggtaatcatgagttcgacaacggggtggaaggtctgatcgatcctctgctccggaatgtgaaatttccaatcctgtcagcaaacattaaggcacgaggaccactggcacaccagatcagcggtctgttcctcccctccaaagtgctgtctgtcgggggcgaggtggtcggcattgtgggatacacctctaaggaaacacccttcctgagtaatcctggcactaacctcgtgtttgaggacgaaatcagtgctctgcagcccgaggtggataagctgaaaaccctcaatgtcaacaagatcattgctctggggcactctggtttcgaaatggacaagctgatcgcacagaaagtgagaggcgtcgatattgtggtcggcggacatagtaatactttcctgtacaccggcaaccccccttcaaaggaggtgccagccggaaaatatccctttatcgtgaccgctgacgatggacggcaggtccctgtggtccaggcctacgctttcggcaagtacctgggatatctcaaagtggagtttgacgataagggcaacgtcattacatcctatggaaatcccatcctgctcaacagctccattcctgaagacgctactatcaaagcagatattaatcagtggaggatcaagctggacaactactccactcaggagctggggagaaccatcgtgtacctggatggctctacccagacatgcaggttcagagaatgtaatatgggcaacctgatctgcgacgccatgattaacaataacctgcgacacccagatgagatgttttggaatcatgtgagcatgtgcatcgtcaacgggggtggcatcaggtcccctattgacgagaagaataacggaactattacctgggaaaacctggccgctgtgctcccattcggagggacatttgatctggtgcagctcaaggggagcactctgaagaaagccttcgagcactcagtgcatcgctacgggcagagcacaggtgaatttctgcaagtgggtggcatccacgtggtctatgacattaatcgaaaaccatggaacagggtggtccagctggaggtgctctgcaccaagtgtcgagtcccaatctacgagcccctggaaatggacaaggtgtacaaagtcacactgcccagctatctcgccaacggaggggatggattccagatgattaaggacgagctgctcaaacatgattctggggaccaggatatctccgtggtctctgagtacattagtaagatgaaagtggtctatccagctgtggaaggcaggatcaagttcgctagcggtggaggagcaggaggtggagctggagggggtgcaggcggaggggccggtggcggaaccggtactcagaacaagcctctgccagagaacgtgaagtacgggatcgtcctggacgccggttctagtcacaccaatctctacatctacaagtggcccgctgagaaagaaaacgatacaggcgtggtccagcagctggaggaatgccaggtgaaggggcctggtatctctaagtacgcccagaaaaccgacgagattggagcttatctggcagagtgtatggaactgtccaccgaactcatcccaacatctaagcaccatcagacacccgtgtacctgggagcaactgcaggaatgcgactgctccgcatggagagtgaacagtcagctgacgaggtgctggcagccgtcagtacttcactcaaaagctatcccttcgattttcagggcgcaaagatcattaccggacaggaggaaggcgcctacggatggatcactattaactatctgctcgggaggttcacccaggagcagagctggctgtccctcatcagcgactcccagaagcaggaaacattcggcgctctggatctcgggggtgcatctactcagatcacctttgtgcctcagaatagtactattgagtcaccagaaaacagcctgcagttcagactctacggcgaggactacacagtgtatactcacagctttctgtgctatggaaaggaccaggccctgtggcagaagctcgctaaagatatccaggtgtcaagcggcggagtcctgaaagatccttgcttcaatccagggtacgagaaggtggtcaacgtgtccgaactgtatggcaccccctgtacaaagaggttcgagaagaaactgcctttcgaccagtttcgaatccagggcaccggagattacgagcagtgtcaccagtctattctggaactcttcaataactcccattgcccctattctcagtgtgccttcaacggcgtgtttctgccacccctccacgggagtttcggtgccttttcagctttctactttgtgatggacttctttaagaaagtggctaagaattctgtcatcagtcaggagaagatgactgaaattaccaagaacttctgctctaaaagttgggaggaaaccaagacatcatatcctagcgtgaaggagaaatacctgagcgaatattgtttttccggagcctacatcctgtccctgctccaggggtataatttcacagactcctcttgggagcagatccacttcatgggcaagatcaaggatagcaacgcagggtggaccctgggttacatgctgaatctcacaaacatgatcccagccgaacagcccctgtcccctccactgcctcactccacctaa

SEQ ID NO: 53 - protein, 1273 aa, Artificial
  Fc-tagged CD73-39 fusion protein derived from mus musculus
MGWSCIILFLVATATGVHSDKTHTCPPCPAPELLGGPSVFLFPPKPKDTLMISRTPEVTCVVVDVSHEDPEVKFNWYVDGVEVHNAKTKPREEQYNSTYRVVSVLTVLHQDWLNGKEYKCKVSNKALPAPIEKTISKAKGQPREPQVYTLPPSREEMTKNQVSLTCLVKGFYPSDIAVEWESNGQPENNYKTTPPVLDSDGSFFLYSKLTVDKSRWQQGNVFSCSVMHEALHNHYTQKSLSLSPGKAAANSSIDLISVPVDSRRPACKIPNDLKQKVMNHDYKDDDDKEWELTILHTNDVHSRLEQTSDDSTKCLNASLCVGGVARLFTKVQQIRKEEPNVLFLDAGDQYQGTIWFTVYKGLEVAHFMNILGYDAMALGNHEFDNGVEGLIDPLLRNVKFPILSANIKARGPLAHQISGLFLPSKVLSVGGEVVGIVGYTSKETPFLSNPGTNLVFEDEISALQPEVDKLKTLNVNKIIALGHSGFEMDKLIAQKVRGVDIVVGGHSNTFLYTGNPPSKEVPAGKYPFIVTADDGRQVPVVQAYAFGKYLGYLKVEFDDKGNVITSYGNPILLNSSIPEDATIKADINQWRIKLDNYSTQELGRTIVYLDGSTQTCRFRECNMGNLICDAMINNNLRHPDEMFWNHVSMCIVNGGGIRSPIDEKNNGTITWENLAAVLPFGGTFDLVQLKGSTLKKAFEHSVHRYGQSTGEFLQVGGIHVVYDINRKPWNRVVQLEVLCTKCRVPIYEPLEMDKVYKVTLPSYLANGGDGFQMIKDELLKHDSGDQDISVVSEYISKMKVVYPAVEGRIKFASGGGAGGGAGGGAGGGAGGGTGTQNKPLPENVKYGIVLDAGSSHTNLYIYKWPAEKENDTGVVQQLEECQVKGPGISKYAQKTDEIGAYLAECMELSTELIPTSKHHQTPVYLGATAGMRLLRMESEQSADEVLAAVSTSLKSYPFDFQGAKIITGQEEGAYGWITINYLLGRFTQEQSWLSLISDSQKQETFGALDLGGASTQITFVPQNSTIESPENSLQFRLYGEDYTVYTHSFLCYGKDQALWQKLAKDIQVSSGGVLKDPCFNPGYEKVVNVSELYGTPCTKRFEKKLPFDQFRIQGTGDYEQCHQSILELFNNSHCPYSQCAFNGVFLPPLHGSFGAFSAFYFVMDFFKKVAKNSVISQEKMTEITKNFCSKSWEETKTSYPSVKEKYLSEYCFSGAYILSLLQGYNFTDSSWEQIHFMGKIKDSNAGWTLGYMLNLTNMIPAEQPLSPPLPHST

SEQ ID NO: 54 - DNA, 3330 bp, Artificial
  CD39-2A-CD73 derived from mus musculus, codon optimized
atgagccgcatggaggacatcaaagactcaaaagtgaaaagattctgctcaaaaaacattctcatcattctggggtttacatcaattctcgctgtgatcgcactgattgccgtcggcctcactcagaacaagcccctgcctgagaacgtgaagtacggaatcgtcctggacgctgggagctcccacaccaatctgtacatctacaagtggccagcagagaaagaaaacgatacaggcgtggtccagcagctggaggaatgccaggtgaagggtcccggcatctccaagtacgcccagaaaacagacgagattggagcttatctggcagagtgtatggaactgagcacagaactcatccccacttccaagcaccatcagacacccgtgtacctgggtgcaactgcaggaatgcgactgctccgcatggagtcagaacagagcgccgacgaggtgctggcagctgtcagtacttcactcaaatcttatccattcgattttcagggtgccaagatcattaccggccaggaggaaggagcttacgggtggatcactattaactatctgctcgggcggttcacccaggagcagtcctggctgtctctcatcagcgactcccagaagcaggaaaccttcggcgctctggatctcggcggagcaagcacccagatcacatttgtgccacagaatagcacaattgagtcccccgaaaactctctgcagttccgcctctacggggaggactacaccgtgtacacccactcctttctgtgctatggcaaggaccaggccctgtggcagaagctcgctaaagatatccaggtgtctagtgggggtgtcctgaaagatccctgcttcaatcctggttacgagaaggtggtcaacgtgtctgaactgtatggaacaccatgtactaagaggttcgagaagaaactgcccttcgaccagtttcgaatccagggaaccggggattacgagcagtgtcaccagagcattctggaactcttcaacaatagccattgcccatattcccagtgtgccttcaacggagtgtttctgccccctctccacggttctttcggcgcctttagtgctttctactttgtgatggacttctttaagaaagtggctaagaatagtgtcatctcacaggagaagatgaccgaaatcacaaagaacttctgctctaagagttgggaggaaaccaagacaagctacccctccgtgaaggagaaatacctgtcagaatattgttttagcggtgcctacatcctgtccctgctccagggctataatttcaccgactcaagctgggagcagatccactttatgggcaagatcaaggattctaacgccggatggaccctggggtacatgctgaatctcacaaacatgatcccagctgagcagccactgtccccaccactccctcattctacctatattggcctgatggtgctcttctccctgctcctggtggctgtcgcaatcacaggactgttcatctactctaagccaagttatttttggaaagaggcagtgggtagtggcgccacaaatttttcactcctgaagcaggccggagacgtggaggaaaacccagggcccatgaggcctgcagccgctaaggtgccaaaatggctcctgctcgcactgtccgccctgctccctcagtggccagcagcctctgcttgggagctgactatcctccacaccaatgatgtgcatagtagactggaacagacctcagacgatagcacaaagtgcctgaacgccagcctgtgcgtgggaggagtcgcaagactgttcaccaaggtgcagcagatccggaaagaggaacctaatgtcctgtttctcgacgcaggcgaccagtaccagggcacaatctggttcaccgtgtacaagggactggaggtcgctcactttatgaacattctgggttacgacgccatggctctcggcaatcatgagttcgacaacggagtggaagggctgatcgatcctctgctccggaatgtgaaatttccaatcctgtcagctaacattaaggcacgaggtcctctggcacaccagatcagcggactgttcctcccaagtaaagtgctgtcagtcgggggcgaggtggtcggtattgtgggctacacctctaaggaaacacccttcctgagtaatcctggcacaaacctcgtgtttgaggacgaaatctctgccctgcagcctgaggtggataagctgaaaactctcaatgtcaacaagatcattgcactgggacacagcgggttcgaaatggacaagctgatcgcccagaaagtgagaggggtcgatattgtggtcggcggacatagtaatactttcctgtacaccggaaaccctccatcaaaggaggtgccagctgggaaatatccctttatcgtgaccgcagacgatggccggcaggtcccagtggtccaggcatacgccttcggcaagtacctgggctatctcaaagtggagtttgacgataagggaaacgtcatcacaagctatgggaatcccatcctgctcaactcctctattcctgaagacgccactatcaaagctgatattaatcagtggaggatcaagctggacaactactccactcaggagctgggaagaaccatcgtgtacctggatgggtctactcagacctgcaggttcagagaatgtaatatgggcaacctgatctgcgacgccatgattaacaataacctgcgacaccccgatgagatgttttggaatcatgtgagcatgtgcatcgtcaacgggggtggcatcaggtcccccattgacgagaagaataacggaacaattacttgggaaaacctggctgcagtgctccctttcggagggacatttgatctggtccagctcaaggggtccactctgaagaaagccttcgagcactcagtgcatcgctacggacagagcaccggggaatttctgcaagtgggtggcatccacgtggtctatgacattaatcgaaaaccctggaacagggtggtccagctggaggtgctctgcactaagtgtcgagtccctatctacgagccactggaaatggacaaggtgtacaaagtcaccctgcctagctatctcgccaacggaggggatggattccagatgattaaggacgagctgctcaaacatgattctggggaccaggatatctccgtggtctctgagtacattagtaagatgaaagtggtctatcctgctgtggaaggcaggatcaagttcagtgccgcttcacattaccagggttcttttccactcgtgattctctctttttgggctatgattctgattctctaa

SEQ ID NO: 55 - DNA, 1533 bp, Artificial
  CD39 cDNA derived from homo sapiens, codon optimized
atggaagataccaaagagagcaacgtgaagactttctgtagcaagaacatcctcgcaatcctggggtttagcagcatcatcgccgtcatcgcactgctcgccgtgggcctcacccagaacaaggccctgcctgagaatgtgaaatacggcattgtcctggacgctggaagctcccacaccagcctgtacatctataagtggcctgctgagaaagaaaacgatacaggggtggtccatcaggtggaggaatgccgggtcaaggggccaggtatttccaagttcgtgcagaaagtcaatgagatcggcatctacctgacagactgtatggagagggctagagaagtgatccctaggtctcagcaccaggaaactccagtctatctgggagcaaccgctggtatgcgactgctccgcatggagagtgaggaactcgcagaccgagtgctggatgtggtcgaaaggtctctgagtaactaccccttcgactttcagggggcacgcatcattactggtcaggaggaaggggcctacggttggatcaccattaattatctgctcggcaagttttctcagaaaacccgatggttcagtattgtgccttatgagacaaacaatcaggaaacttttggagccctcgatctgggcggagcttccacccaggtgacattcgtcccccagaaccagactatcgagtctcctgacaatgccctccagtttaggctgtacgggaaggattacaacgtgtatacccactctttcctgtgctatggtaaagaccaggcactctggcagaagctggccaaagatattcaggtggctagcaacgagatcctgagagacccatgctttcatcccggatacaagaaagtggtcaatgtctccgatctgtataagactccatgtaccaaacggttcgagatgacactgcccttccagcagtttgaaatccagggcattggaaactaccagcagtgtcatcagtctattctcgagctgtttaacactagttactgcccatattcacagtgtgctttcaatggaatctttctcccccctctgcagggcgatttcggagcttttagcgcattctactttgtgatgaagtttctcaatctgacctccgagaaggtgtctcaggagaaagtcacagaaatgatgaagaaattctgcgctcagccctgggaggaaattaagactagctatgcaggggtgaaggagaaatacctgagcgaatattgtttctccggcacatacatcctgtcactgctcctgcagggatatcactttactgccgacagctgggagcacatccatttcattggcaagatccagggatccgatgcagggtggacactgggttacatgctcaacctgactaatatgatccctgccgaacagccactcagtacccccctgtcacatagcacatacgtgttcctgatggtcctgttttcactcgtgctgttcacagtcgctatcattggtctgctcatttttcacaagccctcttatttctggaaggacatggtctga

SEQ ID NO: 56 - DNA, 1725 bp, Artificial
  CD73 cDNA derived from homo sapiens, codon optimized
atgtgccctagagccgctagagcccccgcaaccctcctcctcgccctcggtgctgtcctgtggcccgccgctggtgcttgggaactgactatcctccacaccaatgacgtgcattcacggctggagcagaccagcgaagatagctccaaatgcgtgaacgctagccgctgtatgggcggagtcgcacgactgttcacaaaggtgcagcagatcaggagagccgagcctaatgtgctgctcctggacgctggcgaccagtaccagggcacaatttggttcactgtctataagggagccgaagtggctcactttatgaacgcactccgatacgacgcaatggcactggggaatcatgagttcgataacggagtggaggggctgatcgaacccctcctgaaggaagccaaatttcctatcctctccgcaaacattaaggccaaaggaccactggctagtcagatcagcgggctctacctgccctataaagtcctgcctgtgggcgacgaggtggtcggtattgtgggctatacctccaaggaaacaccattcctctctaatcccggaaccaacctggtgtttgaggacgaaatcacagccctgcagcccgaggtcgataagctcaaaaccctgaatgtgaacaagatcattgctctcggacacagtgggtttgaaatggacaagctgattgcacagaaagtccggggagtggatgtggtcgtggggggtcatagcaatactttcctgtacaccggaaaccccccttccaaggaggtgcctgctgggaaatatcccttcatcgtcacatccgacgatgggaggaaggtgcctgtcgtgcaggcttacgccttcggcaagtacctcggctatctgaaaatcgagtttgacgaaagaggaaatgtgatttctagtcacgggaatccaatcctcctgaactcaagcattccagaggacccctcaatcaaagccgatattaataagtggaggatcaaactggacaactacagcacacaggagctcggcaagactatcgtgtacctggatggctcctctcagtcttgccggttccgcgaatgtaatatgggaaacctgatctgcgacgcaatgattaacaataacctgagacacgccgatgagaccttttggaatcacgtgagcatgtgcatcctgaacggcggagggatcagaagtccaattgacgagcggaataacgggaccattacatgggaaaacctcgcagctgtcctgcccttcggtggcacttttgatctcgtgcagctgaagggcagcaccctgaagaaagccttcgagcacagtgtgcatcgatacggacagtcaactggggaatttctgcaagtgggagggatccacgtcgtgtatgacctgtcccgaaagcccggcgacagggtcgtgaaactcgatgtcctgtgcacaaagtgtcgcgtgccttcttacgacccactgaagatggatgaggtctataaagtgatcctccctaatttcctggcaaacggtggcgatggttttcagatgatcaaggacgaactcctgcggcacgattctggcgaccaggatattaacgtcgtgtctacatacatcagtaagatgaaagtgatctacccagctgtggagggtcgcatcaagttcagcactggctcccattgccacgggtcattttccctcattttcctctccctgtgggcagtcatttttgtcctgtatcagtga

SEQ ID NO: 57 - DNA, 3320 bp, artificial
  CD39-2A-CD73 derived from homo sapiens, codon optimized
atggaggacaccaaggagagcaacgtgaagaccttctgcagcaagaacatcctggccatcctgggcttcagcagcatcatcgccgtgatcgccctgctggccgtgggcctgacccagaacaaggccctgcccgagaacgtgaagtacggcatcgtgctggacgccggcagcagccacaccagcctgtacatctacaagtggcccgccgagaaggagaacgacaccggcgtggtgcaccaggtggaggagtgcagagtgaagggccccggcatcagcaagttcgtgcagaaggtgaacgagatcggcatctacctgaccgactgcatggagagagccagagaggtgatccccagaagccagcaccaggagacccccgtgtacctgggcgccaccgccggcatgagactgctgagaatggagagcgaggagctggccgacagagtgctggacgtggtggagagaagcctgagcaactaccccttcgacttccagggcgccagaatcatcaccggccaggaggagggcgcctacggctggatcaccatcaactacctgctgggcaagttcagccagaagaccagatggttcagcatcgtgccctacgagaccaacaaccaggagaccttcggcgccctggacctgggcggcgccagcacccaggtgaccttcgtgccccagaaccagaccatcgagagccccgacaacgccctgcagttcagactgtacggcaaggactacaacgtgtacacccacagcttcctgtgctacggcaaggaccaggccctgtggcagaagctggccaaggacatccaggtggccagcaacgagatcctgagagacccctgcttccaccccggctacaagaaggtggtgaacgtgagcgacctgtacaagaccccctgcaccaagagattcgagatgaccctgcccttccagcagttcgagatccagggcatcggcaactaccagcagtgccaccagagcatcctggagctgttcaacaccagctactgcccctacagccagtgcgccttcaacggcatcttcctgccccccctgcagggcgacttcggcgccttcagcgccttctacttcgtgatgaagttcctgaacctgaccagcgagaaggtgagccaggagaaggtgaccgagatgatgaagaagttctgcgcccagccctgggaggagatcaagaccagctacgccggcgtgaaggagaagtacctgagcgagtactgcttcagcggcacctacatcctgagcctgctgctgcagggctaccacttcaccgccgacagctgggagcacatccacttcatcggcaagatccagggcagcgacgccggctggaccctgggctacatgctgaacctgaccaacatgatccccgccgagcagcccctgagcacccccctgagccacagcacctacgtgttcctgatggtgctgttcagcctggtgctgttcaccgtggccatcatcggcctgctgatcttccacaagcccagctacttctggaaggacatggtgggcagcggcgccaccaacttcagcctgctgaagcaggccggcgacgtggaggagaaccccggccccatgtgccccagagccgccagagcccccgccaccctgctgctggccctgggcgccgtgctgtggcccgccgccggcgcctgggagctgaccatcctgcacaccaacgacgtgcacagcagactggagcagaccagcgaggacagcagcaagtgcgtgaacgccagcagatgcatgggcggcgtggccagactgttcaccaaggtgcagcagatcagaagagccgagcccaacgtgctgctgctggacgccggcgaccagtaccagggcaccatctggttcaccgtgtacaagggcgccgaggtggcccacttcatgaacgccctgagatacgacgccatggccctgggcaaccacgagttcgacaacggcgtggagggcctgatcgagcccctgctgaaggaggccaagttccccatcctgagcgccaacatcaaggccaagggccccctggccagccagatcagcggcctgtacctgccctacaaggtgctgcccgtgggcgacgaggtggtgggcatcgtgggctacaccagcaaggagacccccttcctgagcaaccccggcaccaacctggtgttcgaggacgagatcaccgccctgcagcccgaggtggacaagctgaagaccctgaacgtgaacaagatcatcgccctgggccacagcggcttcgagatggacaagctgatcgcccagaaggtgagaggcgtggacgtggtggtgggcggccacagcaacaccttcctgtacaccggcaacccccccagcaaggaggtgcccgccggcaagtaccccttcatcgtgaccgcgacgacggcagaaaggtgcccgtggtgcaggcctacgccttcggcaagtacctgggctacctgaagatcgagttcgacgagagaggcaacgtgatcagcagccacggcaaccccatcctgctgaacagcagcatccccgaggaccccagcatcaaggccgacatcaacaagtggagaatcaagctggacaactacagcacccaggagctgggcaagaccatcgtgtacctggacggcagcagccagagctgcagattcagagagtgcaacatgggcaacctgatctgcgacgccatgatcaacaacaacctgagacacgccgacgagaccttctggaaccacgtgagcatgtgcatcctgaacggcggcggcatcagaagccccatcgacgagagaaacaacggcaccatcacctgggagaacctggccgccgtgctgcccttcggcggcaccttcgacctggtgcagctgaagggcagcaccctgaagaaggccttcgagcacagcgtgcacagatacggccagagcaccggcgagttcctgcaggtgggcggcatccacgtggtgtacgacctgagcagaaagcccggcgacagagtggtgaagctggacgtgctgtgcaccaagtgcagagtgcccagctacgaccccctgaagatggacgaggtgtacaaggtgatcctgcccaacttcctggccaacggcggcgacggcttccagatgatcaaggacgagctgctgagacacgacagcggcgaccaggacatcaacgtggtgagcacctacatcagcaagatgaaggtgatctaccccgccgtggagggcagaatcaagttcagcaccggcagccactgccacggcagcttcagcctgatcttcctgagcctgtgggccgtgatcttcgtgctgtaccagtag